European Patent Application EP 4 807 002 A1, published September 16, 2026. Title: 一种抑制甲状腺素转运蛋白(TTR)表达的RNAi 试剂、组合物及应用. Applicant: 成都倍特药业股份有限公司. Application WO. The sequence listing filed with the application follows.

SEQUENCE LISTING (915 sequences)

SEQ ID NO: 1 - RNA, 21 nt, synthetic construct
  source 1..21: mol_type = other RNA
attcttggcaggatggcttct

SEQ ID NO: 2 - RNA, 23 nt, synthetic construct
  source 1..23: mol_type = other RNA
agaagccatcctgccaagaatga

SEQ ID NO: 3 - RNA, 21 nt, synthetic construct
  source 1..21: mol_type = other RNA
ttcttggcaggatggcttcta

SEQ ID NO: 4 - RNA, 23 nt, synthetic construct
  source 1..23: mol_type = other RNA
tagaagccatcctgccaagaatg

SEQ ID NO: 5 - RNA, 21 nt, synthetic construct
  source 1..21: mol_type = other RNA
tcttggcaggatggcttctca

SEQ ID NO: 6 - RNA, 23 nt, synthetic construct
  source 1..23: mol_type = other RNA
tgagaagccatcctgccaagaat

SEQ ID NO: 7 - RNA, 21 nt, synthetic construct
  source 1..21: mol_type = other RNA
cttggcaggatggcttctcat

SEQ ID NO: 8 - RNA, 23 nt, synthetic construct
  source 1..23: mol_type = other RNA
atgagaagccatcctgccaagaa

SEQ ID NO: 9 - RNA, 21 nt, synthetic construct
  source 1..21: mol_type = other RNA
ttggcaggatggcttctcata

SEQ ID NO: 10 - RNA, 23 nt, synthetic construct
  source 1..23: mol_type = other RNA
tatgagaagccatcctgccaaga

SEQ ID NO: 11 - RNA, 21 nt, synthetic construct
  source 1..21: mol_type = other RNA
tggcaggatggcttctcatca

SEQ ID NO: 12 - RNA, 23 nt, synthetic construct
  source 1..23: mol_type = other RNA
tgatgagaagccatcctgccaag

SEQ ID NO: 13 - RNA, 21 nt, synthetic construct
  source 1..21: mol_type = other RNA
ggcaggatggcttctcatcgt

SEQ ID NO: 14 - RNA, 23 nt, synthetic construct
  source 1..23: mol_type = other RNA
acgatgagaagccatcctgccaa

SEQ ID NO: 15 - RNA, 21 nt, synthetic construct
  source 1..21: mol_type = other RNA
gcaggatggcttctcatcgta

SEQ ID NO: 16 - RNA, 23 nt, synthetic construct
  source 1..23: mol_type = other RNA
tacgatgagaagccatcctgcca

SEQ ID NO: 17 - RNA, 21 nt, synthetic construct
  source 1..21: mol_type = other RNA
caggatggcttctcatcgtct

SEQ ID NO: 18 - RNA, 23 nt, synthetic construct
  source 1..23: mol_type = other RNA
agacgatgagaagccatcctgcc

SEQ ID NO: 19 - RNA, 21 nt, synthetic construct
  source 1..21: mol_type = other RNA
aggatggcttctcatcgtcta

SEQ ID NO: 20 - RNA, 23 nt, synthetic construct
  source 1..23: mol_type = other RNA
tagacgatgagaagccatcctgc

SEQ ID NO: 21 - RNA, 21 nt, synthetic construct
  source 1..21: mol_type = other RNA
ggatggcttctcatcgtctga

SEQ ID NO: 22 - RNA, 23 nt, synthetic construct
  source 1..23: mol_type = other RNA
tcagacgatgagaagccatcctg

SEQ ID NO: 23 - RNA, 21 nt, synthetic construct
  source 1..21: mol_type = other RNA
atggcttctcatcgtctgcta

SEQ ID NO: 24 - RNA, 23 nt, synthetic construct
  source 1..23: mol_type = other RNA
tagcagacgatgagaagccatcc

SEQ ID NO: 25 - RNA, 21 nt, synthetic construct
  source 1..21: mol_type = other RNA
tggcttctcatcgtctgctca

SEQ ID NO: 26 - RNA, 23 nt, synthetic construct
  source 1..23: mol_type = other RNA
tgagcagacgatgagaagccatc

SEQ ID NO: 27 - RNA, 21 nt, synthetic construct
  source 1..21: mol_type = other RNA
gcttctcatcgtctgctccta

SEQ ID NO: 28 - RNA, 23 nt, synthetic construct
  source 1..23: mol_type = other RNA
taggagcagacgatgagaagcca

SEQ ID NO: 29 - RNA, 21 nt, synthetic construct
  source 1..21: mol_type = other RNA
tctcatcgtctgctcctccta

SEQ ID NO: 30 - RNA, 23 nt, synthetic construct
  source 1..23: mol_type = other RNA
taggaggagcagacgatgagaag

SEQ ID NO: 31 - RNA, 21 nt, synthetic construct
  source 1..21: mol_type = other RNA
tcatcgtctgctcctcctcta

SEQ ID NO: 32 - RNA, 23 nt, synthetic construct
  source 1..23: mol_type = other RNA
tagaggaggagcagacgatgaga

SEQ ID NO: 33 - RNA, 21 nt, synthetic construct
  source 1..21: mol_type = other RNA
catcgtctgctcctcctctga

SEQ ID NO: 34 - RNA, 23 nt, synthetic construct
  source 1..23: mol_type = other RNA
tcagaggaggagcagacgatgag

SEQ ID NO: 35 - RNA, 21 nt, synthetic construct
  source 1..21: mol_type = other RNA
cgtctgctcctcctctgcctt

SEQ ID NO: 36 - RNA, 23 nt, synthetic construct
  source 1..23: mol_type = other RNA
aaggcagaggaggagcagacgat

SEQ ID NO: 37 - RNA, 21 nt, synthetic construct
  source 1..21: mol_type = other RNA
tgctggactggtatttgtgta

SEQ ID NO: 38 - RNA, 23 nt, synthetic construct
  source 1..23: mol_type = other RNA
tacacaaataccagtccagcaag

SEQ ID NO: 39 - RNA, 21 nt, synthetic construct
  source 1..21: mol_type = other RNA
gctggactggtatttgtgtct

SEQ ID NO: 40 - RNA, 23 nt, synthetic construct
  source 1..23: mol_type = other RNA
agacacaaataccagtccagcaa

SEQ ID NO: 41 - RNA, 21 nt, synthetic construct
  source 1..21: mol_type = other RNA
ctggactggtatttgtgtcta

SEQ ID NO: 42 - RNA, 23 nt, synthetic construct
  source 1..23: mol_type = other RNA
tagacacaaataccagtccagca

SEQ ID NO: 43 - RNA, 21 nt, synthetic construct
  source 1..21: mol_type = other RNA
tggactggtatttgtgtctga

SEQ ID NO: 44 - RNA, 23 nt, synthetic construct
  source 1..23: mol_type = other RNA
tcagacacaaataccagtccagc

SEQ ID NO: 45 - RNA, 21 nt, synthetic construct
  source 1..21: mol_type = other RNA
ggactggtatttgtgtctgaa

SEQ ID NO: 46 - RNA, 23 nt, synthetic construct
  source 1..23: mol_type = other RNA
ttcagacacaaataccagtccag

SEQ ID NO: 47 - RNA, 21 nt, synthetic construct
  source 1..21: mol_type = other RNA
gactggtatttgtgtctgaga

SEQ ID NO: 48 - RNA, 23 nt, synthetic construct
  source 1..23: mol_type = other RNA
tctcagacacaaataccagtcca

SEQ ID NO: 49 - RNA, 21 nt, synthetic construct
  source 1..21: mol_type = other RNA
actggtatttgtgtctgagga

SEQ ID NO: 50 - RNA, 23 nt, synthetic construct
  source 1..23: mol_type = other RNA
tcctcagacacaaataccagtcc

SEQ ID NO: 51 - RNA, 21 nt, synthetic construct
  source 1..21: mol_type = other RNA
tggtatttgtgtctgaggcta

SEQ ID NO: 52 - RNA, 23 nt, synthetic construct
  source 1..23: mol_type = other RNA
tagcctcagacacaaataccagt

SEQ ID NO: 53 - RNA, 21 nt, synthetic construct
  source 1..21: mol_type = other RNA
gtatttgtgtctgaggctgga

SEQ ID NO: 54 - RNA, 23 nt, synthetic construct
  source 1..23: mol_type = other RNA
tccagcctcagacacaaatacca

SEQ ID NO: 55 - RNA, 21 nt, synthetic construct
  source 1..21: mol_type = other RNA
gtgaatccaagtgtcctctga

SEQ ID NO: 56 - RNA, 23 nt, synthetic construct
  source 1..23: mol_type = other RNA
tcagaggacacttggattcaccg

SEQ ID NO: 57 - RNA, 21 nt, synthetic construct
  source 1..21: mol_type = other RNA
tgaatccaagtgtcctctgat

SEQ ID NO: 58 - RNA, 23 nt, synthetic construct
  source 1..23: mol_type = other RNA
atcagaggacacttggattcacc

SEQ ID NO: 59 - RNA, 21 nt, synthetic construct
  source 1..21: mol_type = other RNA
gaatccaagtgtcctctgata

SEQ ID NO: 60 - RNA, 23 nt, synthetic construct
  source 1..23: mol_type = other RNA
tatcagaggacacttggattcac

SEQ ID NO: 61 - RNA, 21 nt, synthetic construct
  source 1..21: mol_type = other RNA
aatccaagtgtcctctgatga

SEQ ID NO: 62 - RNA, 23 nt, synthetic construct
  source 1..23: mol_type = other RNA
tcatcagaggacacttggattca

SEQ ID NO: 63 - RNA, 21 nt, synthetic construct
  source 1..21: mol_type = other RNA
atccaagtgtcctctgatggt

SEQ ID NO: 64 - RNA, 23 nt, synthetic construct
  source 1..23: mol_type = other RNA
accatcagaggacacttggattc

SEQ ID NO: 65 - RNA, 21 nt, synthetic construct
  source 1..21: mol_type = other RNA
tccaagtgtcctctgatggta

SEQ ID NO: 66 - RNA, 23 nt, synthetic construct
  source 1..23: mol_type = other RNA
taccatcagaggacacttggatt

SEQ ID NO: 67 - RNA, 21 nt, synthetic construct
  source 1..21: mol_type = other RNA
ccaagtgtcctctgatggtca

SEQ ID NO: 68 - RNA, 23 nt, synthetic construct
  source 1..23: mol_type = other RNA
tgaccatcagaggacacttggat

SEQ ID NO: 69 - RNA, 21 nt, synthetic construct
  source 1..21: mol_type = other RNA
caagtgtcctctgatggtcaa

SEQ ID NO: 70 - RNA, 23 nt, synthetic construct
  source 1..23: mol_type = other RNA
ttgaccatcagaggacacttgga

SEQ ID NO: 71 - RNA, 21 nt, synthetic construct
  source 1..21: mol_type = other RNA
aagtgtcctctgatggtcaaa

SEQ ID NO: 72 - RNA, 23 nt, synthetic construct
  source 1..23: mol_type = other RNA
tttgaccatcagaggacacttgg

SEQ ID NO: 73 - RNA, 21 nt, synthetic construct
  source 1..21: mol_type = other RNA
agtgtcctctgatggtcaaaa

SEQ ID NO: 74 - RNA, 23 nt, synthetic construct
  source 1..23: mol_type = other RNA
ttttgaccatcagaggacacttg

SEQ ID NO: 75 - RNA, 21 nt, synthetic construct
  source 1..21: mol_type = other RNA
gtgtcctctgatggtcaaagt

SEQ ID NO: 76 - RNA, 23 nt, synthetic construct
  source 1..23: mol_type = other RNA
actttgaccatcagaggacactt

SEQ ID NO: 77 - RNA, 21 nt, synthetic construct
  source 1..21: mol_type = other RNA
tgtcctctgatggtcaaagtt

SEQ ID NO: 78 - RNA, 23 nt, synthetic construct
  source 1..23: mol_type = other RNA
aactttgaccatcagaggacact

SEQ ID NO: 79 - RNA, 21 nt, synthetic construct
  source 1..21: mol_type = other RNA
gtcctctgatggtcaaagtta

SEQ ID NO: 80 - RNA, 23 nt, synthetic construct
  source 1..23: mol_type = other RNA
taactttgaccatcagaggacac

SEQ ID NO: 81 - RNA, 21 nt, synthetic construct
  source 1..21: mol_type = other RNA
tcctctgatggtcaaagttct

SEQ ID NO: 82 - RNA, 23 nt, synthetic construct
  source 1..23: mol_type = other RNA
agaactttgaccatcagaggaca

SEQ ID NO: 83 - RNA, 21 nt, synthetic construct
  source 1..21: mol_type = other RNA
cctctgatggtcaaagttcta

SEQ ID NO: 84 - RNA, 23 nt, synthetic construct
  source 1..23: mol_type = other RNA
tagaactttgaccatcagaggac

SEQ ID NO: 85 - RNA, 21 nt, synthetic construct
  source 1..21: mol_type = other RNA
ctctgatggtcaaagttctaa

SEQ ID NO: 86 - RNA, 23 nt, synthetic construct
  source 1..23: mol_type = other RNA
ttagaactttgaccatcagagga

SEQ ID NO: 87 - RNA, 21 nt, synthetic construct
  source 1..21: mol_type = other RNA
tctgatggtcaaagttctaga

SEQ ID NO: 88 - RNA, 23 nt, synthetic construct
  source 1..23: mol_type = other RNA
tctagaactttgaccatcagagg

SEQ ID NO: 89 - RNA, 21 nt, synthetic construct
  source 1..21: mol_type = other RNA
ctgatggtcaaagttctagat

SEQ ID NO: 90 - RNA, 23 nt, synthetic construct
  source 1..23: mol_type = other RNA
atctagaactttgaccatcagag

SEQ ID NO: 91 - RNA, 21 nt, synthetic construct
  source 1..21: mol_type = other RNA
tgatggtcaaagttctagata

SEQ ID NO: 92 - RNA, 23 nt, synthetic construct
  source 1..23: mol_type = other RNA
tatctagaactttgaccatcaga

SEQ ID NO: 93 - RNA, 21 nt, synthetic construct
  source 1..21: mol_type = other RNA
gatggtcaaagttctagatga

SEQ ID NO: 94 - RNA, 23 nt, synthetic construct
  source 1..23: mol_type = other RNA
tcatctagaactttgaccatcag

SEQ ID NO: 95 - RNA, 21 nt, synthetic construct
  source 1..21: mol_type = other RNA
atggtcaaagttctagatgct

SEQ ID NO: 96 - RNA, 23 nt, synthetic construct
  source 1..23: mol_type = other RNA
agcatctagaactttgaccatca

SEQ ID NO: 97 - RNA, 21 nt, synthetic construct
  source 1..21: mol_type = other RNA
atcaatgtggccgtgcatgta

SEQ ID NO: 98 - RNA, 23 nt, synthetic construct
  source 1..23: mol_type = other RNA
tacatgcacggccacattgatgg

SEQ ID NO: 99 - RNA, 21 nt, synthetic construct
  source 1..21: mol_type = other RNA
agccatttgcctctgggaaaa

SEQ ID NO: 100 - RNA, 23 nt, synthetic construct
  source 1..23: mol_type = other RNA
ttttcccagaggcaaatggctcc

SEQ ID NO: 101 - RNA, 21 nt, synthetic construct
  source 1..21: mol_type = other RNA
gccatttgcctctgggaaaaa

SEQ ID NO: 102 - RNA, 23 nt, synthetic construct
  source 1..23: mol_type = other RNA
tttttcccagaggcaaatggctc

SEQ ID NO: 103 - RNA, 21 nt, synthetic construct
  source 1..21: mol_type = other RNA
ccatttgcctctgggaaaaca

SEQ ID NO: 104 - RNA, 23 nt, synthetic construct
  source 1..23: mol_type = other RNA
tgttttcccagaggcaaatggct

SEQ ID NO: 105 - RNA, 21 nt, synthetic construct
  source 1..21: mol_type = other RNA
catttgcctctgggaaaacca

SEQ ID NO: 106 - RNA, 23 nt, synthetic construct
  source 1..23: mol_type = other RNA
tggttttcccagaggcaaatggc

SEQ ID NO: 107 - RNA, 21 nt, synthetic construct
  source 1..21: mol_type = other RNA
atttgcctctgggaaaaccaa

SEQ ID NO: 108 - RNA, 23 nt, synthetic construct
  source 1..23: mol_type = other RNA
ttggttttcccagaggcaaatgg

SEQ ID NO: 109 - RNA, 21 nt, synthetic construct
  source 1..21: mol_type = other RNA
tttgcctctgggaaaaccagt

SEQ ID NO: 110 - RNA, 23 nt, synthetic construct
  source 1..23: mol_type = other RNA
actggttttcccagaggcaaatg

SEQ ID NO: 111 - RNA, 21 nt, synthetic construct
  source 1..21: mol_type = other RNA
ttgcctctgggaaaaccagta

SEQ ID NO: 112 - RNA, 23 nt, synthetic construct
  source 1..23: mol_type = other RNA
tactggttttcccagaggcaaat

SEQ ID NO: 113 - RNA, 21 nt, synthetic construct
  source 1..21: mol_type = other RNA
tgcctctgggaaaaccagtga

SEQ ID NO: 114 - RNA, 23 nt, synthetic construct
  source 1..23: mol_type = other RNA
tcactggttttcccagaggcaaa

SEQ ID NO: 115 - RNA, 21 nt, synthetic construct
  source 1..21: mol_type = other RNA
gcctctgggaaaaccagtgaa

SEQ ID NO: 116 - RNA, 23 nt, synthetic construct
  source 1..23: mol_type = other RNA
ttcactggttttcccagaggcaa

SEQ ID NO: 117 - RNA, 21 nt, synthetic construct
  source 1..21: mol_type = other RNA
cctctgggaaaaccagtgagt

SEQ ID NO: 118 - RNA, 23 nt, synthetic construct
  source 1..23: mol_type = other RNA
actcactggttttcccagaggca

SEQ ID NO: 119 - RNA, 21 nt, synthetic construct
  source 1..21: mol_type = other RNA
ctctgggaaaaccagtgagta

SEQ ID NO: 120 - RNA, 23 nt, synthetic construct
  source 1..23: mol_type = other RNA
tactcactggttttcccagaggc

SEQ ID NO: 121 - RNA, 21 nt, synthetic construct
  source 1..21: mol_type = other RNA
tctgggaaaaccagtgagtct

SEQ ID NO: 122 - RNA, 23 nt, synthetic construct
  source 1..23: mol_type = other RNA
agactcactggttttcccagagg

SEQ ID NO: 123 - RNA, 21 nt, synthetic construct
  source 1..21: mol_type = other RNA
ctgggaaaaccagtgagtcta

SEQ ID NO: 124 - RNA, 23 nt, synthetic construct
  source 1..23: mol_type = other RNA
tagactcactggttttcccagag

SEQ ID NO: 125 - RNA, 21 nt, synthetic construct
  source 1..21: mol_type = other RNA
tgggaaaaccagtgagtctga

SEQ ID NO: 126 - RNA, 23 nt, synthetic construct
  source 1..23: mol_type = other RNA
tcagactcactggttttcccaga

SEQ ID NO: 127 - RNA, 21 nt, synthetic construct
  source 1..21: mol_type = other RNA
gggaaaaccagtgagtctgga

SEQ ID NO: 128 - RNA, 23 nt, synthetic construct
  source 1..23: mol_type = other RNA
tccagactcactggttttcccag

SEQ ID NO: 129 - RNA, 21 nt, synthetic construct
  source 1..21: mol_type = other RNA
ggaaaaccagtgagtctggaa

SEQ ID NO: 130 - RNA, 23 nt, synthetic construct
  source 1..23: mol_type = other RNA
ttccagactcactggttttccca

SEQ ID NO: 131 - RNA, 21 nt, synthetic construct
  source 1..21: mol_type = other RNA
gaaaaccagtgagtctggaga

SEQ ID NO: 132 - RNA, 23 nt, synthetic construct
  source 1..23: mol_type = other RNA
tctccagactcactggttttccc

SEQ ID NO: 133 - RNA, 21 nt, synthetic construct
  source 1..21: mol_type = other RNA
aaaaccagtgagtctggagaa

SEQ ID NO: 134 - RNA, 23 nt, synthetic construct
  source 1..23: mol_type = other RNA
ttctccagactcactggttttcc

SEQ ID NO: 135 - RNA, 21 nt, synthetic construct
  source 1..21: mol_type = other RNA
aaaccagtgagtctggagaga

SEQ ID NO: 136 - RNA, 23 nt, synthetic construct
  source 1..23: mol_type = other RNA
tctctccagactcactggttttc

SEQ ID NO: 137 - RNA, 21 nt, synthetic construct
  source 1..21: mol_type = other RNA
accagtgagtctggagagcta

SEQ ID NO: 138 - RNA, 23 nt, synthetic construct
  source 1..23: mol_type = other RNA
tagctctccagactcactggttt

SEQ ID NO: 139 - RNA, 21 nt, synthetic construct
  source 1..21: mol_type = other RNA
ccagtgagtctggagagctga

SEQ ID NO: 140 - RNA, 23 nt, synthetic construct
  source 1..23: mol_type = other RNA
tcagctctccagactcactggtt

SEQ ID NO: 141 - RNA, 21 nt, synthetic construct
  source 1..21: mol_type = other RNA
agtgagtctggagagctgcat

SEQ ID NO: 142 - RNA, 23 nt, synthetic construct
  source 1..23: mol_type = other RNA
atgcagctctccagactcactgg

SEQ ID NO: 143 - RNA, 21 nt, synthetic construct
  source 1..21: mol_type = other RNA
gtgagtctggagagctgcata

SEQ ID NO: 144 - RNA, 23 nt, synthetic construct
  source 1..23: mol_type = other RNA
tatgcagctctccagactcactg

SEQ ID NO: 145 - RNA, 21 nt, synthetic construct
  source 1..21: mol_type = other RNA
tgagtctggagagctgcatga

SEQ ID NO: 146 - RNA, 23 nt, synthetic construct
  source 1..23: mol_type = other RNA
tcatgcagctctccagactcact

SEQ ID NO: 147 - RNA, 21 nt, synthetic construct
  source 1..21: mol_type = other RNA
gagtctggagagctgcatgga

SEQ ID NO: 148 - RNA, 23 nt, synthetic construct
  source 1..23: mol_type = other RNA
tccatgcagctctccagactcac

SEQ ID NO: 149 - RNA, 21 nt, synthetic construct
  source 1..21: mol_type = other RNA
tctggagagctgcatgggcta

SEQ ID NO: 150 - RNA, 23 nt, synthetic construct
  source 1..23: mol_type = other RNA
tagcccatgcagctctccagact

SEQ ID NO: 151 - RNA, 21 nt, synthetic construct
  source 1..21: mol_type = other RNA
gagagctgcatgggctcacaa

SEQ ID NO: 152 - RNA, 23 nt, synthetic construct
  source 1..23: mol_type = other RNA
ttgtgagcccatgcagctctcca

SEQ ID NO: 153 - RNA, 21 nt, synthetic construct
  source 1..21: mol_type = other RNA
agagctgcatgggctcacaaa

SEQ ID NO: 154 - RNA, 23 nt, synthetic construct
  source 1..23: mol_type = other RNA
tttgtgagcccatgcagctctcc

SEQ ID NO: 155 - RNA, 21 nt, synthetic construct
  source 1..21: mol_type = other RNA
gagctgcatgggctcacaact

SEQ ID NO: 156 - RNA, 23 nt, synthetic construct
  source 1..23: mol_type = other RNA
agttgtgagcccatgcagctctc

SEQ ID NO: 157 - RNA, 21 nt, synthetic construct
  source 1..21: mol_type = other RNA
agctgcatgggctcacaacta

SEQ ID NO: 158 - RNA, 23 nt, synthetic construct
  source 1..23: mol_type = other RNA
tagttgtgagcccatgcagctct

SEQ ID NO: 159 - RNA, 21 nt, synthetic construct
  source 1..21: mol_type = other RNA
gctgcatgggctcacaactga

SEQ ID NO: 160 - RNA, 23 nt, synthetic construct
  source 1..23: mol_type = other RNA
tcagttgtgagcccatgcagctc

SEQ ID NO: 161 - RNA, 21 nt, synthetic construct
  source 1..21: mol_type = other RNA
ctgcatgggctcacaactgaa

SEQ ID NO: 162 - RNA, 23 nt, synthetic construct
  source 1..23: mol_type = other RNA
ttcagttgtgagcccatgcagct

SEQ ID NO: 163 - RNA, 21 nt, synthetic construct
  source 1..21: mol_type = other RNA
tgcatgggctcacaactgaga

SEQ ID NO: 164 - RNA, 23 nt, synthetic construct
  source 1..23: mol_type = other RNA
tctcagttgtgagcccatgcagc

SEQ ID NO: 165 - RNA, 21 nt, synthetic construct
  source 1..21: mol_type = other RNA
gcatgggctcacaactgagga

SEQ ID NO: 166 - RNA, 23 nt, synthetic construct
  source 1..23: mol_type = other RNA
tcctcagttgtgagcccatgcag

SEQ ID NO: 167 - RNA, 21 nt, synthetic construct
  source 1..21: mol_type = other RNA
catgggctcacaactgaggaa

SEQ ID NO: 168 - RNA, 23 nt, synthetic construct
  source 1..23: mol_type = other RNA
ttcctcagttgtgagcccatgca

SEQ ID NO: 169 - RNA, 21 nt, synthetic construct
  source 1..21: mol_type = other RNA
atgggctcacaactgaggaga

SEQ ID NO: 170 - RNA, 23 nt, synthetic construct
  source 1..23: mol_type = other RNA
tctcctcagttgtgagcccatgc

SEQ ID NO: 171 - RNA, 21 nt, synthetic construct
  source 1..21: mol_type = other RNA
gggctcacaactgaggaggaa

SEQ ID NO: 172 - RNA, 23 nt, synthetic construct
  source 1..23: mol_type = other RNA
ttcctcctcagttgtgagcccat

SEQ ID NO: 173 - RNA, 21 nt, synthetic construct
  source 1..21: mol_type = other RNA
ggctcacaactgaggaggaat

SEQ ID NO: 174 - RNA, 23 nt, synthetic construct
  source 1..23: mol_type = other RNA
attcctcctcagttgtgagccca

SEQ ID NO: 175 - RNA, 21 nt, synthetic construct
  source 1..21: mol_type = other RNA
gctcacaactgaggaggaatt

SEQ ID NO: 176 - RNA, 23 nt, synthetic construct
  source 1..23: mol_type = other RNA
aattcctcctcagttgtgagccc

SEQ ID NO: 177 - RNA, 21 nt, synthetic construct
  source 1..21: mol_type = other RNA
ctcacaactgaggaggaattt

SEQ ID NO: 178 - RNA, 23 nt, synthetic construct
  source 1..23: mol_type = other RNA
aaattcctcctcagttgtgagcc

SEQ ID NO: 179 - RNA, 21 nt, synthetic construct
  source 1..21: mol_type = other RNA
tcacaactgaggaggaattta

SEQ ID NO: 180 - RNA, 23 nt, synthetic construct
  source 1..23: mol_type = other RNA
taaattcctcctcagttgtgagc

SEQ ID NO: 181 - RNA, 21 nt, synthetic construct
  source 1..21: mol_type = other RNA
cacaactgaggaggaatttgt

SEQ ID NO: 182 - RNA, 23 nt, synthetic construct
  source 1..23: mol_type = other RNA
acaaattcctcctcagttgtgag

SEQ ID NO: 183 - RNA, 21 nt, synthetic construct
  source 1..21: mol_type = other RNA
acaactgaggaggaatttgta

SEQ ID NO: 184 - RNA, 23 nt, synthetic construct
  source 1..23: mol_type = other RNA
tacaaattcctcctcagttgtga

SEQ ID NO: 185 - RNA, 21 nt, synthetic construct
  source 1..21: mol_type = other RNA
caactgaggaggaatttgtaa

SEQ ID NO: 186 - RNA, 23 nt, synthetic construct
  source 1..23: mol_type = other RNA
ttacaaattcctcctcagttgtg

SEQ ID NO: 187 - RNA, 21 nt, synthetic construct
  source 1..21: mol_type = other RNA
aactgaggaggaatttgtaga

SEQ ID NO: 188 - RNA, 23 nt, synthetic construct
  source 1..23: mol_type = other RNA
tctacaaattcctcctcagttgt

SEQ ID NO: 189 - RNA, 21 nt, synthetic construct
  source 1..21: mol_type = other RNA
actgaggaggaatttgtagaa

SEQ ID NO: 190 - RNA, 23 nt, synthetic construct
  source 1..23: mol_type = other RNA
ttctacaaattcctcctcagttg

SEQ ID NO: 191 - RNA, 21 nt, synthetic construct
  source 1..21: mol_type = other RNA
ctgaggaggaatttgtagaaa

SEQ ID NO: 192 - RNA, 23 nt, synthetic construct
  source 1..23: mol_type = other RNA
tttctacaaattcctcctcagtt

SEQ ID NO: 193 - RNA, 21 nt, synthetic construct
  source 1..21: mol_type = other RNA
tgaggaggaatttgtagaaga

SEQ ID NO: 194 - RNA, 23 nt, synthetic construct
  source 1..23: mol_type = other RNA
tcttctacaaattcctcctcagt

SEQ ID NO: 195 - RNA, 21 nt, synthetic construct
  source 1..21: mol_type = other RNA
gaggaggaatttgtagaagga

SEQ ID NO: 196 - RNA, 23 nt, synthetic construct
  source 1..23: mol_type = other RNA
tccttctacaaattcctcctcag

SEQ ID NO: 197 - RNA, 21 nt, synthetic construct
  source 1..21: mol_type = other RNA
aggaggaatttgtagaaggga

SEQ ID NO: 198 - RNA, 23 nt, synthetic construct
  source 1..23: mol_type = other RNA
tcccttctacaaattcctcctca

SEQ ID NO: 199 - RNA, 21 nt, synthetic construct
  source 1..21: mol_type = other RNA
ggaggaatttgtagaagggat

SEQ ID NO: 200 - RNA, 23 nt, synthetic construct
  source 1..23: mol_type = other RNA
atcccttctacaaattcctcctc

SEQ ID NO: 201 - RNA, 21 nt, synthetic construct
  source 1..21: mol_type = other RNA
gaggaatttgtagaagggata

SEQ ID NO: 202 - RNA, 23 nt, synthetic construct
  source 1..23: mol_type = other RNA
tatcccttctacaaattcctcct

SEQ ID NO: 203 - RNA, 21 nt, synthetic construct
  source 1..21: mol_type = other RNA
aggaatttgtagaagggatat

SEQ ID NO: 204 - RNA, 23 nt, synthetic construct
  source 1..23: mol_type = other RNA
atatcccttctacaaattcctcc

SEQ ID NO: 205 - RNA, 21 nt, synthetic construct
  source 1..21: mol_type = other RNA
ggaatttgtagaagggatata

SEQ ID NO: 206 - RNA, 23 nt, synthetic construct
  source 1..23: mol_type = other RNA
tatatcccttctacaaattcctc

SEQ ID NO: 207 - RNA, 21 nt, synthetic construct
  source 1..21: mol_type = other RNA
gaatttgtagaagggatataa

SEQ ID NO: 208 - RNA, 23 nt, synthetic construct
  source 1..23: mol_type = other RNA
ttatatcccttctacaaattcct

SEQ ID NO: 209 - RNA, 21 nt, synthetic construct
  source 1..21: mol_type = other RNA
aatttgtagaagggatataca

SEQ ID NO: 210 - RNA, 23 nt, synthetic construct
  source 1..23: mol_type = other RNA
tgtatatcccttctacaaattcc

SEQ ID NO: 211 - RNA, 21 nt, synthetic construct
  source 1..21: mol_type = other RNA
atttgtagaagggatatacaa

SEQ ID NO: 212 - RNA, 23 nt, synthetic construct
  source 1..23: mol_type = other RNA
ttgtatatcccttctacaaattc

SEQ ID NO: 213 - RNA, 21 nt, synthetic construct
  source 1..21: mol_type = other RNA
tttgtagaagggatatacaaa

SEQ ID NO: 214 - RNA, 23 nt, synthetic construct
  source 1..23: mol_type = other RNA
tttgtatatcccttctacaaatt

SEQ ID NO: 215 - RNA, 21 nt, synthetic construct
  source 1..21: mol_type = other RNA
ttgtagaagggatatacaaaa

SEQ ID NO: 216 - RNA, 23 nt, synthetic construct
  source 1..23: mol_type = other RNA
ttttgtatatcccttctacaaat

SEQ ID NO: 217 - RNA, 21 nt, synthetic construct
  source 1..21: mol_type = other RNA
tgtagaagggatatacaaagt

SEQ ID NO: 218 - RNA, 23 nt, synthetic construct
  source 1..23: mol_type = other RNA
actttgtatatcccttctacaaa

SEQ ID NO: 219 - RNA, 21 nt, synthetic construct
  source 1..21: mol_type = other RNA
gtagaagggatatacaaagta

SEQ ID NO: 220 - RNA, 23 nt, synthetic construct
  source 1..23: mol_type = other RNA
tactttgtatatcccttctacaa

SEQ ID NO: 221 - RNA, 21 nt, synthetic construct
  source 1..21: mol_type = other RNA
tagaagggatatacaaagtga

SEQ ID NO: 222 - RNA, 23 nt, synthetic construct
  source 1..23: mol_type = other RNA
tcactttgtatatcccttctaca

SEQ ID NO: 223 - RNA, 21 nt, synthetic construct
  source 1..21: mol_type = other RNA
agaagggatatacaaagtgga

SEQ ID NO: 224 - RNA, 23 nt, synthetic construct
  source 1..23: mol_type = other RNA
tccactttgtatatcccttctac

SEQ ID NO: 225 - RNA, 21 nt, synthetic construct
  source 1..21: mol_type = other RNA
gaagggatatacaaagtggaa

SEQ ID NO: 226 - RNA, 23 nt, synthetic construct
  source 1..23: mol_type = other RNA
ttccactttgtatatcccttcta

SEQ ID NO: 227 - RNA, 21 nt, synthetic construct
  source 1..21: mol_type = other RNA
aagggatatacaaagtggaaa

SEQ ID NO: 228 - RNA, 23 nt, synthetic construct
  source 1..23: mol_type = other RNA
tttccactttgtatatcccttct

SEQ ID NO: 229 - RNA, 21 nt, synthetic construct
  source 1..21: mol_type = other RNA
agggatatacaaagtggaaat

SEQ ID NO: 230 - RNA, 23 nt, synthetic construct
  source 1..23: mol_type = other RNA
atttccactttgtatatcccttc

SEQ ID NO: 231 - RNA, 21 nt, synthetic construct
  source 1..21: mol_type = other RNA
gggatatacaaagtggaaata

SEQ ID NO: 232 - RNA, 23 nt, synthetic construct
  source 1..23: mol_type = other RNA
tatttccactttgtatatccctt

SEQ ID NO: 233 - RNA, 21 nt, synthetic construct
  source 1..21: mol_type = other RNA
ggatatacaaagtggaaataa

SEQ ID NO: 234 - RNA, 23 nt, synthetic construct
  source 1..23: mol_type = other RNA
ttatttccactttgtatatccct

SEQ ID NO: 235 - RNA, 21 nt, synthetic construct
  source 1..21: mol_type = other RNA
gatatacaaagtggaaataga

SEQ ID NO: 236 - RNA, 23 nt, synthetic construct
  source 1..23: mol_type = other RNA
tctatttccactttgtatatccc

SEQ ID NO: 237 - RNA, 21 nt, synthetic construct
  source 1..21: mol_type = other RNA
atatacaaagtggaaatagaa

SEQ ID NO: 238 - RNA, 23 nt, synthetic construct
  source 1..23: mol_type = other RNA
ttctatttccactttgtatatcc

SEQ ID NO: 239 - RNA, 21 nt, synthetic construct
  source 1..21: mol_type = other RNA
tatacaaagtggaaatagaca

SEQ ID NO: 240 - RNA, 23 nt, synthetic construct
  source 1..23: mol_type = other RNA
tgtctatttccactttgtatatc

SEQ ID NO: 241 - RNA, 21 nt, synthetic construct
  source 1..21: mol_type = other RNA
atacaaagtggaaatagacaa

SEQ ID NO: 242 - RNA, 23 nt, synthetic construct
  source 1..23: mol_type = other RNA
ttgtctatttccactttgtatat

SEQ ID NO: 243 - RNA, 21 nt, synthetic construct
  source 1..21: mol_type = other RNA
tacaaagtggaaatagacaca

SEQ ID NO: 244 - RNA, 23 nt, synthetic construct
  source 1..23: mol_type = other RNA
tgtgtctatttccactttgtata

SEQ ID NO: 245 - RNA, 21 nt, synthetic construct
  source 1..21: mol_type = other RNA
acaaagtggaaatagacacca

SEQ ID NO: 246 - RNA, 23 nt, synthetic construct
  source 1..23: mol_type = other RNA
tggtgtctatttccactttgtat

SEQ ID NO: 247 - RNA, 21 nt, synthetic construct
  source 1..21: mol_type = other RNA
caaagtggaaatagacaccaa

SEQ ID NO: 248 - RNA, 23 nt, synthetic construct
  source 1..23: mol_type = other RNA
ttggtgtctatttccactttgta

SEQ ID NO: 249 - RNA, 21 nt, synthetic construct
  source 1..21: mol_type = other RNA
aaagtggaaatagacaccaaa

SEQ ID NO: 250 - RNA, 23 nt, synthetic construct
  source 1..23: mol_type = other RNA
tttggtgtctatttccactttgt

SEQ ID NO: 251 - RNA, 21 nt, synthetic construct
  source 1..21: mol_type = other RNA
aagtggaaatagacaccaaat

SEQ ID NO: 252 - RNA, 23 nt, synthetic construct
  source 1..23: mol_type = other RNA
atttggtgtctatttccactttg

SEQ ID NO: 253 - RNA, 21 nt, synthetic construct
  source 1..21: mol_type = other RNA
agtggaaatagacaccaaata

SEQ ID NO: 254 - RNA, 23 nt, synthetic construct
  source 1..23: mol_type = other RNA
tatttggtgtctatttccacttt

SEQ ID NO: 255 - RNA, 21 nt, synthetic construct
  source 1..21: mol_type = other RNA
gtggaaatagacaccaaatct

SEQ ID NO: 256 - RNA, 23 nt, synthetic construct
  source 1..23: mol_type = other RNA
agatttggtgtctatttccactt

SEQ ID NO: 257 - RNA, 21 nt, synthetic construct
  source 1..21: mol_type = other RNA
tggaaatagacaccaaatctt

SEQ ID NO: 258 - RNA, 23 nt, synthetic construct
  source 1..23: mol_type = other RNA
aagatttggtgtctatttccact

SEQ ID NO: 259 - RNA, 21 nt, synthetic construct
  source 1..21: mol_type = other RNA
ggaaatagacaccaaatctta

SEQ ID NO: 260 - RNA, 23 nt, synthetic construct
  source 1..23: mol_type = other RNA
taagatttggtgtctatttccac

SEQ ID NO: 261 - RNA, 21 nt, synthetic construct
  source 1..21: mol_type = other RNA
gaaatagacaccaaatcttaa

SEQ ID NO: 262 - RNA, 23 nt, synthetic construct
  source 1..23: mol_type = other RNA
ttaagatttggtgtctatttcca

SEQ ID NO: 263 - RNA, 21 nt, synthetic construct
  source 1..21: mol_type = other RNA
aaatagacaccaaatcttact

SEQ ID NO: 264 - RNA, 23 nt, synthetic construct
  source 1..23: mol_type = other RNA
agtaagatttggtgtctatttcc

SEQ ID NO: 265 - RNA, 21 nt, synthetic construct
  source 1..21: mol_type = other RNA
aatagacaccaaatcttacta

SEQ ID NO: 266 - RNA, 23 nt, synthetic construct
  source 1..23: mol_type = other RNA
tagtaagatttggtgtctatttc

SEQ ID NO: 267 - RNA, 21 nt, synthetic construct
  source 1..21: mol_type = other RNA
atagacaccaaatcttactga

SEQ ID NO: 268 - RNA, 23 nt, synthetic construct
  source 1..23: mol_type = other RNA
tcagtaagatttggtgtctattt

SEQ ID NO: 269 - RNA, 21 nt, synthetic construct
  source 1..21: mol_type = other RNA
tagacaccaaatcttactgga

SEQ ID NO: 270 - RNA, 23 nt, synthetic construct
  source 1..23: mol_type = other RNA
tccagtaagatttggtgtctatt

SEQ ID NO: 271 - RNA, 21 nt, synthetic construct
  source 1..21: mol_type = other RNA
agacaccaaatcttactggaa

SEQ ID NO: 272 - RNA, 23 nt, synthetic construct
  source 1..23: mol_type = other RNA
ttccagtaagatttggtgtctat

SEQ ID NO: 273 - RNA, 21 nt, synthetic construct
  source 1..21: mol_type = other RNA
gacaccaaatcttactggaaa

SEQ ID NO: 274 - RNA, 23 nt, synthetic construct
  source 1..23: mol_type = other RNA
tttccagtaagatttggtgtcta

SEQ ID NO: 275 - RNA, 21 nt, synthetic construct
  source 1..21: mol_type = other RNA
gcacttggcatctccccatta

SEQ ID NO: 276 - RNA, 23 nt, synthetic construct
  source 1..23: mol_type = other RNA
taatggggagatgccaagtgcct

SEQ ID NO: 277 - RNA, 21 nt, synthetic construct
  source 1..21: mol_type = other RNA
cacttggcatctccccattca

SEQ ID NO: 278 - RNA, 23 nt, synthetic construct
  source 1..23: mol_type = other RNA
tgaatggggagatgccaagtgcc

SEQ ID NO: 279 - RNA, 21 nt, synthetic construct
  source 1..21: mol_type = other RNA
acttggcatctccccattcca

SEQ ID NO: 280 - RNA, 23 nt, synthetic construct
  source 1..23: mol_type = other RNA
tggaatggggagatgccaagtgc

SEQ ID NO: 281 - RNA, 21 nt, synthetic construct
  source 1..21: mol_type = other RNA
cttggcatctccccattccat

SEQ ID NO: 282 - RNA, 23 nt, synthetic construct
  source 1..23: mol_type = other RNA
atggaatggggagatgccaagtg

SEQ ID NO: 283 - RNA, 21 nt, synthetic construct
  source 1..21: mol_type = other RNA
ttggcatctccccattccata

SEQ ID NO: 284 - RNA, 23 nt, synthetic construct
  source 1..23: mol_type = other RNA
tatggaatggggagatgccaagt

SEQ ID NO: 285 - RNA, 21 nt, synthetic construct
  source 1..21: mol_type = other RNA
tggcatctccccattccatga

SEQ ID NO: 286 - RNA, 23 nt, synthetic construct
  source 1..23: mol_type = other RNA
tcatggaatggggagatgccaag

SEQ ID NO: 287 - RNA, 21 nt, synthetic construct
  source 1..21: mol_type = other RNA
ggcatctccccattccatgaa

SEQ ID NO: 288 - RNA, 23 nt, synthetic construct
  source 1..23: mol_type = other RNA
ttcatggaatggggagatgccaa

SEQ ID NO: 289 - RNA, 21 nt, synthetic construct
  source 1..21: mol_type = other RNA
gcatctccccattccatgaga

SEQ ID NO: 290 - RNA, 23 nt, synthetic construct
  source 1..23: mol_type = other RNA
tctcatggaatggggagatgcca

SEQ ID NO: 291 - RNA, 21 nt, synthetic construct
  source 1..21: mol_type = other RNA
catctccccattccatgagca

SEQ ID NO: 292 - RNA, 23 nt, synthetic construct
  source 1..23: mol_type = other RNA
tgctcatggaatggggagatgcc

SEQ ID NO: 293 - RNA, 21 nt, synthetic construct
  source 1..21: mol_type = other RNA
atctccccattccatgagcat

SEQ ID NO: 294 - RNA, 23 nt, synthetic construct
  source 1..23: mol_type = other RNA
atgctcatggaatggggagatgc

SEQ ID NO: 295 - RNA, 21 nt, synthetic construct
  source 1..21: mol_type = other RNA
tctccccattccatgagcata

SEQ ID NO: 296 - RNA, 23 nt, synthetic construct
  source 1..23: mol_type = other RNA
tatgctcatggaatggggagatg

SEQ ID NO: 297 - RNA, 21 nt, synthetic construct
  source 1..21: mol_type = other RNA
ctccccattccatgagcatga

SEQ ID NO: 298 - RNA, 23 nt, synthetic construct
  source 1..23: mol_type = other RNA
tcatgctcatggaatggggagat

SEQ ID NO: 299 - RNA, 21 nt, synthetic construct
  source 1..21: mol_type = other RNA
tccccattccatgagcatgca

SEQ ID NO: 300 - RNA, 23 nt, synthetic construct
  source 1..23: mol_type = other RNA
tgcatgctcatggaatggggaga

SEQ ID NO: 301 - RNA, 21 nt, synthetic construct
  source 1..21: mol_type = other RNA
ccccattccatgagcatgcaa

SEQ ID NO: 302 - RNA, 23 nt, synthetic construct
  source 1..23: mol_type = other RNA
ttgcatgctcatggaatggggag

SEQ ID NO: 303 - RNA, 21 nt, synthetic construct
  source 1..21: mol_type = other RNA
cccattccatgagcatgcaga

SEQ ID NO: 304 - RNA, 23 nt, synthetic construct
  source 1..23: mol_type = other RNA
tctgcatgctcatggaatgggga

SEQ ID NO: 305 - RNA, 21 nt, synthetic construct
  source 1..21: mol_type = other RNA
ccattccatgagcatgcagaa

SEQ ID NO: 306 - RNA, 23 nt, synthetic construct
  source 1..23: mol_type = other RNA
ttctgcatgctcatggaatgggg

SEQ ID NO: 307 - RNA, 21 nt, synthetic construct
  source 1..21: mol_type = other RNA
cattccatgagcatgcagaga

SEQ ID NO: 308 - RNA, 23 nt, synthetic construct
  source 1..23: mol_type = other RNA
tctctgcatgctcatggaatggg

SEQ ID NO: 309 - RNA, 21 nt, synthetic construct
  source 1..21: mol_type = other RNA
ttccatgagcatgcagaggta

SEQ ID NO: 310 - RNA, 23 nt, synthetic construct
  source 1..23: mol_type = other RNA
tacctctgcatgctcatggaatg

SEQ ID NO: 311 - RNA, 21 nt, synthetic construct
  source 1..21: mol_type = other RNA
tccatgagcatgcagaggtga

SEQ ID NO: 312 - RNA, 23 nt, synthetic construct
  source 1..23: mol_type = other RNA
tcacctctgcatgctcatggaat

SEQ ID NO: 313 - RNA, 21 nt, synthetic construct
  source 1..21: mol_type = other RNA
catgagcatgcagaggtggta

SEQ ID NO: 314 - RNA, 23 nt, synthetic construct
  source 1..23: mol_type = other RNA
taccacctctgcatgctcatgga

SEQ ID NO: 315 - RNA, 21 nt, synthetic construct
  source 1..21: mol_type = other RNA
atgagcatgcagaggtggtat

SEQ ID NO: 316 - RNA, 23 nt, synthetic construct
  source 1..23: mol_type = other RNA
ataccacctctgcatgctcatgg

SEQ ID NO: 317 - RNA, 21 nt, synthetic construct
  source 1..21: mol_type = other RNA
tgagcatgcagaggtggtatt

SEQ ID NO: 318 - RNA, 23 nt, synthetic construct
  source 1..23: mol_type = other RNA
aataccacctctgcatgctcatg

SEQ ID NO: 319 - RNA, 21 nt, synthetic construct
  source 1..21: mol_type = other RNA
gagcatgcagaggtggtatta

SEQ ID NO: 320 - RNA, 23 nt, synthetic construct
  source 1..23: mol_type = other RNA
taataccacctctgcatgctcat

SEQ ID NO: 321 - RNA, 21 nt, synthetic construct
  source 1..21: mol_type = other RNA
agcatgcagaggtggtattca

SEQ ID NO: 322 - RNA, 23 nt, synthetic construct
  source 1..23: mol_type = other RNA
tgaataccacctctgcatgctca

SEQ ID NO: 323 - RNA, 21 nt, synthetic construct
  source 1..21: mol_type = other RNA
gcatgcagaggtggtattcaa

SEQ ID NO: 324 - RNA, 23 nt, synthetic construct
  source 1..23: mol_type = other RNA
ttgaataccacctctgcatgctc

SEQ ID NO: 325 - RNA, 21 nt, synthetic construct
  source 1..21: mol_type = other RNA
catgcagaggtggtattcaca

SEQ ID NO: 326 - RNA, 23 nt, synthetic construct
  source 1..23: mol_type = other RNA
tgtgaataccacctctgcatgct

SEQ ID NO: 327 - RNA, 21 nt, synthetic construct
  source 1..21: mol_type = other RNA
atgcagaggtggtattcacaa

SEQ ID NO: 328 - RNA, 23 nt, synthetic construct
  source 1..23: mol_type = other RNA
ttgtgaataccacctctgcatgc

SEQ ID NO: 329 - RNA, 21 nt, synthetic construct
  source 1..21: mol_type = other RNA
tgcagaggtggtattcacaga

SEQ ID NO: 330 - RNA, 23 nt, synthetic construct
  source 1..23: mol_type = other RNA
tctgtgaataccacctctgcatg

SEQ ID NO: 331 - RNA, 21 nt, synthetic construct
  source 1..21: mol_type = other RNA
gcagaggtggtattcacagca

SEQ ID NO: 332 - RNA, 23 nt, synthetic construct
  source 1..23: mol_type = other RNA
tgctgtgaataccacctctgcat

SEQ ID NO: 333 - RNA, 21 nt, synthetic construct
  source 1..21: mol_type = other RNA
agaggtggtattcacagccaa

SEQ ID NO: 334 - RNA, 23 nt, synthetic construct
  source 1..23: mol_type = other RNA
ttggctgtgaataccacctctgc

SEQ ID NO: 335 - RNA, 21 nt, synthetic construct
  source 1..21: mol_type = other RNA
gaggtggtattcacagccaaa

SEQ ID NO: 336 - RNA, 23 nt, synthetic construct
  source 1..23: mol_type = other RNA
tttggctgtgaataccacctctg

SEQ ID NO: 337 - RNA, 21 nt, synthetic construct
  source 1..21: mol_type = other RNA
aggtggtattcacagccaaca

SEQ ID NO: 338 - RNA, 23 nt, synthetic construct
  source 1..23: mol_type = other RNA
tgttggctgtgaataccacctct

SEQ ID NO: 339 - RNA, 21 nt, synthetic construct
  source 1..21: mol_type = other RNA
cctgctgagcccctactccta

SEQ ID NO: 340 - RNA, 23 nt, synthetic construct
  source 1..23: mol_type = other RNA
taggagtaggggctcagcagggc

SEQ ID NO: 341 - RNA, 21 nt, synthetic construct
  source 1..21: mol_type = other RNA
ctgctgagcccctactcctat

SEQ ID NO: 342 - RNA, 23 nt, synthetic construct
  source 1..23: mol_type = other RNA
ataggagtaggggctcagcaggg

SEQ ID NO: 343 - RNA, 21 nt, synthetic construct
  source 1..21: mol_type = other RNA
tgctgagcccctactcctatt

SEQ ID NO: 344 - RNA, 23 nt, synthetic construct
  source 1..23: mol_type = other RNA
aataggagtaggggctcagcagg

SEQ ID NO: 345 - RNA, 21 nt, synthetic construct
  source 1..21: mol_type = other RNA
gctgagcccctactcctatta

SEQ ID NO: 346 - RNA, 23 nt, synthetic construct
  source 1..23: mol_type = other RNA
taataggagtaggggctcagcag

SEQ ID NO: 347 - RNA, 21 nt, synthetic construct
  source 1..21: mol_type = other RNA
ctgagcccctactcctattca

SEQ ID NO: 348 - RNA, 23 nt, synthetic construct
  source 1..23: mol_type = other RNA
tgaataggagtaggggctcagca

SEQ ID NO: 349 - RNA, 21 nt, synthetic construct
  source 1..21: mol_type = other RNA
tgagcccctactcctattcca

SEQ ID NO: 350 - RNA, 23 nt, synthetic construct
  source 1..23: mol_type = other RNA
tggaataggagtaggggctcagc

SEQ ID NO: 351 - RNA, 21 nt, synthetic construct
  source 1..21: mol_type = other RNA
gagcccctactcctattccaa

SEQ ID NO: 352 - RNA, 23 nt, synthetic construct
  source 1..23: mol_type = other RNA
ttggaataggagtaggggctcag

SEQ ID NO: 353 - RNA, 21 nt, synthetic construct
  source 1..21: mol_type = other RNA
agcccctactcctattccaca

SEQ ID NO: 354 - RNA, 23 nt, synthetic construct
  source 1..23: mol_type = other RNA
tgtggaataggagtaggggctca

SEQ ID NO: 355 - RNA, 21 nt, synthetic construct
  source 1..21: mol_type = other RNA
gcccctactcctattccacca

SEQ ID NO: 356 - RNA, 23 nt, synthetic construct
  source 1..23: mol_type = other RNA
tggtggaataggagtaggggctc

SEQ ID NO: 357 - RNA, 21 nt, synthetic construct
  source 1..21: mol_type = other RNA
cccctactcctattccaccaa

SEQ ID NO: 358 - RNA, 23 nt, synthetic construct
  source 1..23: mol_type = other RNA
ttggtggaataggagtaggggct

SEQ ID NO: 359 - RNA, 21 nt, synthetic construct
  source 1..21: mol_type = other RNA
tattccaccacggctgtcgta

SEQ ID NO: 360 - RNA, 23 nt, synthetic construct
  source 1..23: mol_type = other RNA
tacgacagccgtggtggaatagg

SEQ ID NO: 361 - RNA, 21 nt, synthetic construct
  source 1..21: mol_type = other RNA
attccaccacggctgtcgtca

SEQ ID NO: 362 - RNA, 23 nt, synthetic construct
  source 1..23: mol_type = other RNA
tgacgacagccgtggtggaatag

SEQ ID NO: 363 - RNA, 21 nt, synthetic construct
  source 1..21: mol_type = other RNA
ttccaccacggctgtcgtcaa

SEQ ID NO: 364 - RNA, 23 nt, synthetic construct
  source 1..23: mol_type = other RNA
ttgacgacagccgtggtggaata

SEQ ID NO: 365 - RNA, 21 nt, synthetic construct
  source 1..21: mol_type = other RNA
caccacggctgtcgtcaccaa

SEQ ID NO: 366 - RNA, 23 nt, synthetic construct
  source 1..23: mol_type = other RNA
ttggtgacgacagccgtggtgga

SEQ ID NO: 367 - RNA, 21 nt, synthetic construct
  source 1..21: mol_type = other RNA
accacggctgtcgtcaccaat

SEQ ID NO: 368 - RNA, 23 nt, synthetic construct
  source 1..23: mol_type = other RNA
attggtgacgacagccgtggtgg

SEQ ID NO: 369 - RNA, 21 nt, synthetic construct
  source 1..21: mol_type = other RNA
ccacggctgtcgtcaccaata

SEQ ID NO: 370 - RNA, 23 nt, synthetic construct
  source 1..23: mol_type = other RNA
tattggtgacgacagccgtggtg

SEQ ID NO: 371 - RNA, 21 nt, synthetic construct
  source 1..21: mol_type = other RNA
cacggctgtcgtcaccaatca

SEQ ID NO: 372 - RNA, 23 nt, synthetic construct
  source 1..23: mol_type = other RNA
tgattggtgacgacagccgtggt

SEQ ID NO: 373 - RNA, 21 nt, synthetic construct
  source 1..21: mol_type = other RNA
acggctgtcgtcaccaatcca

SEQ ID NO: 374 - RNA, 23 nt, synthetic construct
  source 1..23: mol_type = other RNA
tggattggtgacgacagccgtgg

SEQ ID NO: 375 - RNA, 21 nt, synthetic construct
  source 1..21: mol_type = other RNA
cggctgtcgtcaccaatccca

SEQ ID NO: 376 - RNA, 23 nt, synthetic construct
  source 1..23: mol_type = other RNA
tgggattggtgacgacagccgtg

SEQ ID NO: 377 - RNA, 21 nt, synthetic construct
  source 1..21: mol_type = other RNA
ggctgtcgtcaccaatcccaa

SEQ ID NO: 378 - RNA, 23 nt, synthetic construct
  source 1..23: mol_type = other RNA
ttgggattggtgacgacagccgt

SEQ ID NO: 379 - RNA, 21 nt, synthetic construct
  source 1..21: mol_type = other RNA
gctgtcgtcaccaatcccaaa

SEQ ID NO: 380 - RNA, 23 nt, synthetic construct
  source 1..23: mol_type = other RNA
tttgggattggtgacgacagccg

SEQ ID NO: 381 - RNA, 21 nt, synthetic construct
  source 1..21: mol_type = other RNA
ctgtcgtcaccaatcccaaga

SEQ ID NO: 382 - RNA, 23 nt, synthetic construct
  source 1..23: mol_type = other RNA
tcttgggattggtgacgacagcc

SEQ ID NO: 383 - RNA, 21 nt, synthetic construct
  source 1..21: mol_type = other RNA
gtcgtcaccaatcccaaggaa

SEQ ID NO: 384 - RNA, 23 nt, synthetic construct
  source 1..23: mol_type = other RNA
ttccttgggattggtgacgacag

SEQ ID NO: 385 - RNA, 21 nt, synthetic construct
  source 1..21: mol_type = other RNA
tcgtcaccaatcccaaggaat

SEQ ID NO: 386 - RNA, 23 nt, synthetic construct
  source 1..23: mol_type = other RNA
attccttgggattggtgacgaca

SEQ ID NO: 387 - RNA, 21 nt, synthetic construct
  source 1..21: mol_type = other RNA
cgtcaccaatcccaaggaata

SEQ ID NO: 388 - RNA, 23 nt, synthetic construct
  source 1..23: mol_type = other RNA
tattccttgggattggtgacgac

SEQ ID NO: 389 - RNA, 21 nt, synthetic construct
  source 1..21: mol_type = other RNA
gtcaccaatcccaaggaatga

SEQ ID NO: 390 - RNA, 23 nt, synthetic construct
  source 1..23: mol_type = other RNA
tcattccttgggattggtgacga

SEQ ID NO: 391 - RNA, 21 nt, synthetic construct
  source 1..21: mol_type = other RNA
tcaccaatcccaaggaatgaa

SEQ ID NO: 392 - RNA, 23 nt, synthetic construct
  source 1..23: mol_type = other RNA
ttcattccttgggattggtgacg

SEQ ID NO: 393 - RNA, 21 nt, synthetic construct
  source 1..21: mol_type = other RNA
caccaatcccaaggaatgaga

SEQ ID NO: 394 - RNA, 23 nt, synthetic construct
  source 1..23: mol_type = other RNA
tctcattccttgggattggtgac

SEQ ID NO: 395 - RNA, 21 nt, synthetic construct
  source 1..21: mol_type = other RNA
accaatcccaaggaatgagga

SEQ ID NO: 396 - RNA, 23 nt, synthetic construct
  source 1..23: mol_type = other RNA
tcctcattccttgggattggtga

SEQ ID NO: 397 - RNA, 21 nt, synthetic construct
  source 1..21: mol_type = other RNA
ccaatcccaaggaatgaggga

SEQ ID NO: 398 - RNA, 23 nt, synthetic construct
  source 1..23: mol_type = other RNA
tccctcattccttgggattggtg

SEQ ID NO: 399 - RNA, 21 nt, synthetic construct
  source 1..21: mol_type = other RNA
caatcccaaggaatgagggaa

SEQ ID NO: 400 - RNA, 23 nt, synthetic construct
  source 1..23: mol_type = other RNA
ttccctcattccttgggattggt

SEQ ID NO: 401 - RNA, 21 nt, synthetic construct
  source 1..21: mol_type = other RNA
atcccaaggaatgagggactt

SEQ ID NO: 402 - RNA, 23 nt, synthetic construct
  source 1..23: mol_type = other RNA
aagtccctcattccttgggattg

SEQ ID NO: 403 - RNA, 21 nt, synthetic construct
  source 1..21: mol_type = other RNA
tcccaaggaatgagggactta

SEQ ID NO: 404 - RNA, 23 nt, synthetic construct
  source 1..23: mol_type = other RNA
taagtccctcattccttgggatt

SEQ ID NO: 405 - RNA, 21 nt, synthetic construct
  source 1..21: mol_type = other RNA
cccaaggaatgagggacttct

SEQ ID NO: 406 - RNA, 23 nt, synthetic construct
  source 1..23: mol_type = other RNA
agaagtccctcattccttgggat

SEQ ID NO: 407 - RNA, 21 nt, synthetic construct
  source 1..21: mol_type = other RNA
ccaaggaatgagggacttcta

SEQ ID NO: 408 - RNA, 23 nt, synthetic construct
  source 1..23: mol_type = other RNA
tagaagtccctcattccttggga

SEQ ID NO: 409 - RNA, 21 nt, synthetic construct
  source 1..21: mol_type = other RNA
caaggaatgagggacttctca

SEQ ID NO: 410 - RNA, 23 nt, synthetic construct
  source 1..23: mol_type = other RNA
tgagaagtccctcattccttggg

SEQ ID NO: 411 - RNA, 21 nt, synthetic construct
  source 1..21: mol_type = other RNA
aaggaatgagggacttctcct

SEQ ID NO: 412 - RNA, 23 nt, synthetic construct
  source 1..23: mol_type = other RNA
aggagaagtccctcattccttgg

SEQ ID NO: 413 - RNA, 21 nt, synthetic construct
  source 1..21: mol_type = other RNA
tgggatttcatgtaaccaaga

SEQ ID NO: 414 - RNA, 23 nt, synthetic construct
  source 1..23: mol_type = other RNA
tcttggttacatgaaatcccatc

SEQ ID NO: 415 - RNA, 21 nt, synthetic construct
  source 1..21: mol_type = other RNA
atgtaaccaagagtattccat

SEQ ID NO: 416 - RNA, 23 nt, synthetic construct
  source 1..23: mol_type = other RNA
atggaatactcttggttacatga

SEQ ID NO: 417 - RNA, 21 nt, synthetic construct
  source 1..21: mol_type = other RNA
ttactaaagcagtgttttcaa

SEQ ID NO: 418 - RNA, 23 nt, synthetic construct
  source 1..23: mol_type = other RNA
ttgaaaacactgctttagtaaaa

SEQ ID NO: 419 - RNA, 21 nt, synthetic construct
  source 1..21: mol_type = other RNA
tactaaagcagtgttttcaca

SEQ ID NO: 420 - RNA, 23 nt, synthetic construct
  source 1..23: mol_type = other RNA
tgtgaaaacactgctttagtaaa

SEQ ID NO: 421 - RNA, 21 nt, synthetic construct
  source 1..21: mol_type = other RNA
actaaagcagtgttttcacct

SEQ ID NO: 422 - RNA, 23 nt, synthetic construct
  source 1..23: mol_type = other RNA
aggtgaaaacactgctttagtaa

SEQ ID NO: 423 - RNA, 21 nt, synthetic construct
  source 1..21: mol_type = other RNA
ctaaagcagtgttttcaccta

SEQ ID NO: 424 - RNA, 23 nt, synthetic construct
  source 1..23: mol_type = other RNA
taggtgaaaacactgctttaggg

SEQ ID NO: 425 - RNA, 21 nt, synthetic construct
  source 1..21: mol_type = other RNA
taaagcagtgttttcacctca

SEQ ID NO: 426 - RNA, 23 nt, synthetic construct
  source 1..23: mol_type = other RNA
tgaggtgaaaacactgctttagt

SEQ ID NO: 427 - RNA, 21 nt, synthetic construct
  source 1..21: mol_type = other RNA
aaagcagtgttttcacctcat

SEQ ID NO: 428 - RNA, 23 nt, synthetic construct
  source 1..23: mol_type = other RNA
atgaggtgaaaacactgctttag

SEQ ID NO: 429 - RNA, 21 nt, synthetic construct
  source 1..21: mol_type = other RNA
aagcagtgttttcacctcata

SEQ ID NO: 430 - RNA, 23 nt, synthetic construct
  source 1..23: mol_type = other RNA
tatgaggtgaaaacactgcttta

SEQ ID NO: 431 - RNA, 21 nt, synthetic construct
  source 1..21: mol_type = other RNA
agcagtgttttcacctcatat

SEQ ID NO: 432 - RNA, 23 nt, synthetic construct
  source 1..23: mol_type = other RNA
atatgaggtgaaaacactgctgg

SEQ ID NO: 433 - RNA, 21 nt, synthetic construct
  source 1..21: mol_type = other RNA
aagtccaggcagagacaataa

SEQ ID NO: 434 - RNA, 23 nt, synthetic construct
  source 1..23: mol_type = other RNA
ttattgtctctgcctggacttct

SEQ ID NO: 435 - RNA, 21 nt, synthetic construct
  source 1..21: mol_type = other RNA
agtccaggcagagacaataaa

SEQ ID NO: 436 - RNA, 23 nt, synthetic construct
  source 1..23: mol_type = other RNA
tttattgtctctgcctggacttc

SEQ ID NO: 437 - RNA, 21 nt, synthetic construct
  source 1..21: mol_type = other RNA
gtccaggcagagacaataaaa

SEQ ID NO: 438 - RNA, 23 nt, synthetic construct
  source 1..23: mol_type = other RNA
ttttattgtctctgcctggactt

SEQ ID NO: 439 - RNA, 21 nt, synthetic construct
  source 1..21: mol_type = other RNA
ccaggcagagacaataaaaca

SEQ ID NO: 440 - RNA, 23 nt, synthetic construct
  source 1..23: mol_type = other RNA
tgttttattgtctctgcctggac

SEQ ID NO: 441 - RNA, 21 nt, synthetic construct
  source 1..21: mol_type = other RNA
caggcagagacaataaaacat

SEQ ID NO: 442 - RNA, 23 nt, synthetic construct
  source 1..23: mol_type = other RNA
atgttttattgtctctgcctgga

SEQ ID NO: 443 - RNA, 21 nt, synthetic construct
  source 1..21: mol_type = other RNA
aggcagagacaataaaacatt

SEQ ID NO: 444 - RNA, 23 nt, synthetic construct
  source 1..23: mol_type = other RNA
aatgttttattgtctctgcctgg

SEQ ID NO: 445 - RNA, 21 nt, synthetic construct
  source 1..21: mol_type = other RNA
ggcagagacaataaaacatta

SEQ ID NO: 446 - RNA, 23 nt, synthetic construct
  source 1..23: mol_type = other RNA
taatgttttattgtctctgcctg

SEQ ID NO: 447 - RNA, 21 nt, synthetic construct
  source 1..21: mol_type = other RNA
gcagagacaataaaacattca

SEQ ID NO: 448 - RNA, 23 nt, synthetic construct
  source 1..23: mol_type = other RNA
tgaatgttttattgtctctgcct

SEQ ID NO: 449 - RNA, 21 nt, synthetic construct
  source 1..21: mol_type = other RNA
cagagacaataaaacattcct

SEQ ID NO: 450 - RNA, 23 nt, synthetic construct
  source 1..23: mol_type = other RNA
aggaatgttttattgtctctgcc

SEQ ID NO: 451 - RNA, 21 nt, synthetic construct
  source 1..21: mol_type = other RNA
agagacaataaaacattccta

SEQ ID NO: 452 - RNA, 23 nt, synthetic construct
  source 1..23: mol_type = other RNA
taggaatgttttattgtctctgc

SEQ ID NO: 453 - RNA, 21 nt, synthetic construct
  source 1..21: mol_type = other RNA
gagacaataaaacattcctgt

SEQ ID NO: 454 - RNA, 23 nt, synthetic construct
  source 1..23: mol_type = other RNA
acaggaatgttttattgtctctg

SEQ ID NO: 455 - RNA, 21 nt, synthetic construct
  source 1..21: mol_type = other RNA
agacaataaaacattcctgta

SEQ ID NO: 456 - RNA, 23 nt, synthetic construct
  source 1..23: mol_type = other RNA
tacaggaatgttttattgtctct

SEQ ID NO: 457 - RNA, 21 nt, synthetic construct
  source 1..21: mol_type = other RNA
gacaataaaacattcctgtga

SEQ ID NO: 458 - RNA, 23 nt, synthetic construct
  source 1..23: mol_type = other RNA
tcacaggaatgttttattgtctc

SEQ ID NO: 459 - RNA, 21 nt, synthetic construct
  source 1..21: mol_type = other RNA
acaataaaacattcctgtgaa

SEQ ID NO: 460 - RNA, 23 nt, synthetic construct
  source 1..23: mol_type = other RNA
ttcacaggaatgttttattgtct

SEQ ID NO: 461 - RNA, 21 nt, synthetic construct
  source 1..21: mol_type = other RNA
caataaaacattcctgtgaaa

SEQ ID NO: 462 - RNA, 23 nt, synthetic construct
  source 1..23: mol_type = other RNA
tttcacaggaatgttttattgtc

SEQ ID NO: 463 - RNA, 21 nt, synthetic construct
  source 1..21: mol_type = other RNA
aataaaacattcctgtgaaaa

SEQ ID NO: 464 - RNA, 23 nt, synthetic construct
  source 1..23: mol_type = other RNA
ttttcacaggaatgttttattgt

SEQ ID NO: 465 - RNA, 21 nt, synthetic construct
  source 1..21: mol_type = other RNA
ataaaacattcctgtgaaaga

SEQ ID NO: 466 - RNA, 23 nt, synthetic construct
  source 1..23: mol_type = other RNA
tctttcacaggaatgttttattg

SEQ ID NO: 467 - RNA, 21 nt, synthetic construct
  source 1..21: mol_type = other RNA
taaaacattcctgtgaaagga

SEQ ID NO: 468 - RNA, 23 nt, synthetic construct
  source 1..23: mol_type = other RNA
tcctttcacaggaatgttttatt

SEQ ID NO: 469 - RNA, 21 nt, synthetic construct
  source 1..21: mol_type = other RNA
aaaacattcctgtgaaaggca

SEQ ID NO: 470 - RNA, 23 nt, synthetic construct
  source 1..23: mol_type = other RNA
tgcctttcacaggaatgttttat

SEQ ID NO: 471 - RNA, 21 nt, synthetic construct
  source 1..21: mol_type = other RNA
tccaagtgtcctctgatggta

SEQ ID NO: 472 - RNA, 21 nt, synthetic construct
  source 1..21: mol_type = other RNA
tccaagtgtcctctgatggta

SEQ ID NO: 473 - RNA, 21 nt, synthetic construct
  source 1..21: mol_type = other RNA
tccaagtgtcctctgatggta

SEQ ID NO: 474 - RNA, 21 nt, synthetic construct
  source 1..21: mol_type = other RNA
tccaagtgtcctctgatggta

SEQ ID NO: 475 - RNA, 21 nt, synthetic construct
  source 1..21: mol_type = other RNA
tccaagtgtcctctgatggta

SEQ ID NO: 476 - RNA, 21 nt, synthetic construct
  source 1..21: mol_type = other RNA
tccaagtgtcctctgatggta

SEQ ID NO: 477 - RNA, 21 nt, synthetic construct
  source 1..21: mol_type = other RNA
tccaagtgtcctctgatggta

SEQ ID NO: 478 - RNA, 21 nt, synthetic construct
  source 1..21: mol_type = other RNA
tccaagtgtcctctgatggta

SEQ ID NO: 479 - RNA, 21 nt, synthetic construct
  source 1..21: mol_type = other RNA
cctctgatggtcaaagttcta

SEQ ID NO: 480 - RNA, 21 nt, synthetic construct
  source 1..21: mol_type = other RNA
cctctgatggtcaaagttcta

SEQ ID NO: 481 - RNA, 21 nt, synthetic construct
  source 1..21: mol_type = other RNA
cctctgatggtcaaagttcta

SEQ ID NO: 482 - RNA, 21 nt, synthetic construct
  source 1..21: mol_type = other RNA
cctctgatggtcaaagttcta

SEQ ID NO: 483 - RNA, 21 nt, synthetic construct
  source 1..21: mol_type = other RNA
cctctgatggtcaaagttcta

SEQ ID NO: 484 - RNA, 21 nt, synthetic construct
  source 1..21: mol_type = other RNA
cctctgatggtcaaagttcta

SEQ ID NO: 485 - RNA, 21 nt, synthetic construct
  source 1..21: mol_type = other RNA
cctctgatggtcaaagttcta

SEQ ID NO: 486 - RNA, 21 nt, synthetic construct
  source 1..21: mol_type = other RNA
cctctgatggtcaaagttcta

SEQ ID NO: 487 - RNA, 21 nt, synthetic construct
  source 1..21: mol_type = other RNA
ctgatggtcaaagttctagat

SEQ ID NO: 488 - RNA, 21 nt, synthetic construct
  source 1..21: mol_type = other RNA
ctgatggtcaaagttctagaa

SEQ ID NO: 489 - RNA, 21 nt, synthetic construct
  source 1..21: mol_type = other RNA
ctgatggtcaaagttctagat

SEQ ID NO: 490 - RNA, 21 nt, synthetic construct
  source 1..21: mol_type = other RNA
ctgatggtcaaagttctagat

SEQ ID NO: 491 - RNA, 21 nt, synthetic construct
  source 1..21: mol_type = other RNA
ctgatggtcaaagttctagaa

SEQ ID NO: 492 - RNA, 21 nt, synthetic construct
  source 1..21: mol_type = other RNA
ctgatggtcaaagttctagat

SEQ ID NO: 493 - RNA, 21 nt, synthetic construct
  source 1..21: mol_type = other RNA
ctgatggtcaaagttctagaa

SEQ ID NO: 494 - RNA, 21 nt, synthetic construct
  source 1..21: mol_type = other RNA
ctgatggtcaaagttctagat

SEQ ID NO: 495 - RNA, 21 nt, synthetic construct
  source 1..21: mol_type = other RNA
ctgatggtcaaagttctagaa

SEQ ID NO: 496 - RNA, 21 nt, synthetic construct
  source 1..21: mol_type = other RNA
ctgatggtcaaagttctagat

SEQ ID NO: 497 - RNA, 21 nt, synthetic construct
  source 1..21: mol_type = other RNA
ctgatggtcaaagttctagaa

SEQ ID NO: 498 - RNA, 21 nt, synthetic construct
  source 1..21: mol_type = other RNA
ctgatggtcaaagttctagat

SEQ ID NO: 499 - RNA, 21 nt, synthetic construct
  source 1..21: mol_type = other RNA
ctgatggtcaaagttctagaa

SEQ ID NO: 500 - RNA, 21 nt, synthetic construct
  source 1..21: mol_type = other RNA
ctgatggtcaaagttctagat

SEQ ID NO: 501 - RNA, 21 nt, synthetic construct
  source 1..21: mol_type = other RNA
gatatacaaagtggaaataga

SEQ ID NO: 502 - RNA, 21 nt, synthetic construct
  source 1..21: mol_type = other RNA
gatatacaaagtggaaataga

SEQ ID NO: 503 - RNA, 21 nt, synthetic construct
  source 1..21: mol_type = other RNA
gatatacaaagtggaaataga

SEQ ID NO: 504 - RNA, 21 nt, synthetic construct
  source 1..21: mol_type = other RNA
gatatacaaagtggaaataga

SEQ ID NO: 505 - RNA, 21 nt, synthetic construct
  source 1..21: mol_type = other RNA
gatatacaaagtggaaataga

SEQ ID NO: 506 - RNA, 21 nt, synthetic construct
  source 1..21: mol_type = other RNA
gatatacaaagtggaaataga

SEQ ID NO: 507 - RNA, 21 nt, synthetic construct
  source 1..21: mol_type = other RNA
gatatacaaagtggaaataga

SEQ ID NO: 508 - RNA, 21 nt, synthetic construct
  source 1..21: mol_type = other RNA
gatatacaaagtggaaataga

SEQ ID NO: 509 - RNA, 21 nt, synthetic construct
  source 1..21: mol_type = other RNA
ggaaatagacaccaaatctta

SEQ ID NO: 510 - RNA, 21 nt, synthetic construct
  source 1..21: mol_type = other RNA
ggaaatagacaccaaatctta

SEQ ID NO: 511 - RNA, 21 nt, synthetic construct
  source 1..21: mol_type = other RNA
ggaaatagacaccaaatctta

SEQ ID NO: 512 - RNA, 21 nt, synthetic construct
  source 1..21: mol_type = other RNA
ggaaatagacaccaaatctta

SEQ ID NO: 513 - RNA, 21 nt, synthetic construct
  source 1..21: mol_type = other RNA
ggaaatagacaccaaatctta

SEQ ID NO: 514 - RNA, 21 nt, synthetic construct
  source 1..21: mol_type = other RNA
ggaaatagacaccaaatctta

SEQ ID NO: 515 - RNA, 21 nt, synthetic construct
  source 1..21: mol_type = other RNA
ggaaatagacaccaaatctta

SEQ ID NO: 516 - RNA, 21 nt, synthetic construct
  source 1..21: mol_type = other RNA
ggaaatagacaccaaatctta

SEQ ID NO: 517 - RNA, 21 nt, synthetic construct
  source 1..21: mol_type = other RNA
atgcagaggtggtattcacaa

SEQ ID NO: 518 - RNA, 21 nt, synthetic construct
  source 1..21: mol_type = other RNA
atgcagaggtggtattcacaa

SEQ ID NO: 519 - RNA, 21 nt, synthetic construct
  source 1..21: mol_type = other RNA
atgcagaggtggtattcacaa

SEQ ID NO: 520 - RNA, 21 nt, synthetic construct
  source 1..21: mol_type = other RNA
atgcagaggtggtattcacaa

SEQ ID NO: 521 - RNA, 21 nt, synthetic construct
  source 1..21: mol_type = other RNA
atgcagaggtggtattcacaa

SEQ ID NO: 522 - RNA, 21 nt, synthetic construct
  source 1..21: mol_type = other RNA
atgcagaggtggtattcacaa

SEQ ID NO: 523 - RNA, 21 nt, synthetic construct
  source 1..21: mol_type = other RNA
atgcagaggtggtattcacaa

SEQ ID NO: 524 - RNA, 21 nt, synthetic construct
  source 1..21: mol_type = other RNA
atgcagaggtggtattcacaa

SEQ ID NO: 525 - RNA, 21 nt, synthetic construct
  source 1..21: mol_type = other RNA
cctgctgagcccctactccta

SEQ ID NO: 526 - RNA, 21 nt, synthetic construct
  source 1..21: mol_type = other RNA
cctgctgagcccctactccta

SEQ ID NO: 527 - RNA, 21 nt, synthetic construct
  source 1..21: mol_type = other RNA
cctgctgagcccctactccta

SEQ ID NO: 528 - RNA, 21 nt, synthetic construct
  source 1..21: mol_type = other RNA
cctgctgagcccctactccta

SEQ ID NO: 529 - RNA, 21 nt, synthetic construct
  source 1..21: mol_type = other RNA
cctgctgagcccctactccta

SEQ ID NO: 530 - RNA, 21 nt, synthetic construct
  source 1..21: mol_type = other RNA
cctgctgagcccctactccta

SEQ ID NO: 531 - RNA, 21 nt, synthetic construct
  source 1..21: mol_type = other RNA
cctgctgagcccctactccta

SEQ ID NO: 532 - RNA, 21 nt, synthetic construct
  source 1..21: mol_type = other RNA
cctgctgagcccctactccta

SEQ ID NO: 533 - RNA, 21 nt, synthetic construct
  source 1..21: mol_type = other RNA
ctaaagcagtgttttcaccta

SEQ ID NO: 534 - RNA, 21 nt, synthetic construct
  source 1..21: mol_type = other RNA
ctaaagcagtgttttcaccta

SEQ ID NO: 535 - RNA, 21 nt, synthetic construct
  source 1..21: mol_type = other RNA
ctaaagcagtgttttcaccta

SEQ ID NO: 536 - RNA, 21 nt, synthetic construct
  source 1..21: mol_type = other RNA
ctaaagcagtgttttcaccta

SEQ ID NO: 537 - RNA, 21 nt, synthetic construct
  source 1..21: mol_type = other RNA
agcagtgttttcacctcatat

SEQ ID NO: 538 - RNA, 21 nt, synthetic construct
  source 1..21: mol_type = other RNA
agcagtgttttcacctcataa

SEQ ID NO: 539 - RNA, 21 nt, synthetic construct
  source 1..21: mol_type = other RNA
agcagtgttttcacctcataa

SEQ ID NO: 540 - RNA, 21 nt, synthetic construct
  source 1..21: mol_type = other RNA
agcagtgttttcacctcatat

SEQ ID NO: 541 - RNA, 21 nt, synthetic construct
  source 1..21: mol_type = other RNA
agcagtgttttcacctcatat

SEQ ID NO: 542 - RNA, 21 nt, synthetic construct
  source 1..21: mol_type = other RNA
gtccaggcagagacaataaaa

SEQ ID NO: 543 - RNA, 21 nt, synthetic construct
  source 1..21: mol_type = other RNA
gtccaggcagagacaataaaa

SEQ ID NO: 544 - RNA, 21 nt, synthetic construct
  source 1..21: mol_type = other RNA
gtccaggcagagacaataaaa

SEQ ID NO: 545 - RNA, 21 nt, synthetic construct
  source 1..21: mol_type = other RNA
gtccaggcagagacaataaaa

SEQ ID NO: 546 - RNA, 21 nt, synthetic construct
  source 1..21: mol_type = other RNA
gtccaggcagagacaataaaa

SEQ ID NO: 547 - RNA, 21 nt, synthetic construct
  source 1..21: mol_type = other RNA
gtccaggcagagacaataaaa

SEQ ID NO: 548 - RNA, 21 nt, synthetic construct
  source 1..21: mol_type = other RNA
gtccaggcagagacaataaaa

SEQ ID NO: 549 - RNA, 21 nt, synthetic construct
  source 1..21: mol_type = other RNA
gtccaggcagagacaataaaa

SEQ ID NO: 550 - RNA, 21 nt, synthetic construct
  source 1..21: mol_type = other RNA
aggcagagacaataaaacatt

SEQ ID NO: 551 - RNA, 21 nt, synthetic construct
  source 1..21: mol_type = other RNA
aggcagagacaataaaacata

SEQ ID NO: 552 - RNA, 21 nt, synthetic construct
  source 1..21: mol_type = other RNA
aggcagagacaataaaacatt

SEQ ID NO: 553 - RNA, 21 nt, synthetic construct
  source 1..21: mol_type = other RNA
aggcagagacaataaaacata

SEQ ID NO: 554 - RNA, 21 nt, synthetic construct
  source 1..21: mol_type = other RNA
aggcagagacaataaaacata

SEQ ID NO: 555 - RNA, 21 nt, synthetic construct
  source 1..21: mol_type = other RNA
aggcagagacaataaaacata

SEQ ID NO: 556 - RNA, 21 nt, synthetic construct
  source 1..21: mol_type = other RNA
aggcagagacaataaaacata

SEQ ID NO: 557 - RNA, 21 nt, synthetic construct
  source 1..21: mol_type = other RNA
aggcagagacaataaaacata

SEQ ID NO: 558 - RNA, 21 nt, synthetic construct
  source 1..21: mol_type = other RNA
aggcagagacaataaaacatt

SEQ ID NO: 559 - RNA, 21 nt, synthetic construct
  source 1..21: mol_type = other RNA
agagacaataaaacattccta

SEQ ID NO: 560 - RNA, 21 nt, synthetic construct
  source 1..21: mol_type = other RNA
agagacaataaaacattccta

SEQ ID NO: 561 - RNA, 21 nt, synthetic construct
  source 1..21: mol_type = other RNA
agagacaataaaacattccta

SEQ ID NO: 562 - RNA, 21 nt, synthetic construct
  source 1..21: mol_type = other RNA
agagacaataaaacattccta

SEQ ID NO: 563 - RNA, 21 nt, synthetic construct
  source 1..21: mol_type = other RNA
agagacaataaaacattccta

SEQ ID NO: 564 - RNA, 21 nt, synthetic construct
  source 1..21: mol_type = other RNA
agagacaataaaacattccta

SEQ ID NO: 565 - RNA, 21 nt, synthetic construct
  source 1..21: mol_type = other RNA
agagacaataaaacattccta

SEQ ID NO: 566 - RNA, 21 nt, synthetic construct
  source 1..21: mol_type = other RNA
agagacaataaaacattccta

SEQ ID NO: 567 - RNA, 21 nt, synthetic construct
  source 1..21: mol_type = other RNA
caataaaacattcctgtgaaa

SEQ ID NO: 568 - RNA, 21 nt, synthetic construct
  source 1..21: mol_type = other RNA
caataaaacattcctgtgaaa

SEQ ID NO: 569 - RNA, 21 nt, synthetic construct
  source 1..21: mol_type = other RNA
caataaaacattcctgtgaaa

SEQ ID NO: 570 - RNA, 21 nt, synthetic construct
  source 1..21: mol_type = other RNA
caataaaacattcctgtgaaa

SEQ ID NO: 571 - RNA, 21 nt, synthetic construct
  source 1..21: mol_type = other RNA
caataaaacattcctgtgaaa

SEQ ID NO: 572 - RNA, 21 nt, synthetic construct
  source 1..21: mol_type = other RNA
caataaaacattcctgtgaaa

SEQ ID NO: 573 - RNA, 21 nt, synthetic construct
  source 1..21: mol_type = other RNA
caataaaacattcctgtgaaa

SEQ ID NO: 574 - RNA, 21 nt, synthetic construct
  source 1..21: mol_type = other RNA
caataaaacattcctgtgaaa

SEQ ID NO: 575 - RNA, 23 nt, synthetic construct
  source 1..23: mol_type = other RNA
taccatcagaggacacttggatt

SEQ ID NO: 576 - RNA, 23 nt, synthetic construct
  source 1..23: mol_type = other RNA
taccatcagaggacacttggatt

SEQ ID NO: 577 - RNA, 23 nt, synthetic construct
  source 1..23: mol_type = other RNA
taccatcagaggacacttggatt

SEQ ID NO: 578 - RNA, 23 nt, synthetic construct
  source 1..23: mol_type = other RNA
taccatcagaggacacttggatt

SEQ ID NO: 579 - RNA, 23 nt, synthetic construct
  source 1..23: mol_type = other RNA
taccatcagaggacacttggatt

SEQ ID NO: 580 - RNA, 23 nt, synthetic construct
  source 1..23: mol_type = other RNA
taccatcagaggacacttggatt

SEQ ID NO: 581 - RNA, 23 nt, synthetic construct
  source 1..23: mol_type = other RNA
taccatcagaggacacttggatt

SEQ ID NO: 582 - RNA, 23 nt, synthetic construct
  source 1..23: mol_type = other RNA
taccatcagaggacacttggatt

SEQ ID NO: 583 - RNA, 23 nt, synthetic construct
  source 1..23: mol_type = other RNA
taccatcagaggacacttggatt

SEQ ID NO: 584 - RNA, 23 nt, synthetic construct
  source 1..23: mol_type = other RNA
taccatcagaggacacttggatt

SEQ ID NO: 585 - RNA, 23 nt, synthetic construct
  source 1..23: mol_type = other RNA
taccatcagaggacacttggatt

SEQ ID NO: 586 - RNA, 23 nt, synthetic construct
  source 1..23: mol_type = other RNA
taccatcagaggacacttggatt

SEQ ID NO: 587 - RNA, 23 nt, synthetic construct
  source 1..23: mol_type = other RNA
taccatcagaggacacttggatt

SEQ ID NO: 588 - RNA, 23 nt, synthetic construct
  source 1..23: mol_type = other RNA
taccatcagaggacacttggatt

SEQ ID NO: 589 - RNA, 23 nt, synthetic construct
  source 1..23: mol_type = other RNA
taccatcagaggacacttggatt

SEQ ID NO: 590 - RNA, 23 nt, synthetic construct
  source 1..23: mol_type = other RNA
taccatcagaggacacttggatt

SEQ ID NO: 591 - RNA, 23 nt, synthetic construct
  source 1..23: mol_type = other RNA
taccatcagaggacacttggatt

SEQ ID NO: 592 - RNA, 23 nt, synthetic construct
  source 1..23: mol_type = other RNA
taccatcagaggacacttggatt

SEQ ID NO: 593 - RNA, 23 nt, synthetic construct
  source 1..23: mol_type = other RNA
taccatcagaggacacttggatt

SEQ ID NO: 594 - RNA, 23 nt, synthetic construct
  source 1..23: mol_type = other RNA
taccatcagaggacacttggatt

SEQ ID NO: 595 - RNA, 23 nt, synthetic construct
  source 1..23: mol_type = other RNA
taccatcagaggacacttggatt

SEQ ID NO: 596 - RNA, 23 nt, synthetic construct
  source 1..23: mol_type = other RNA
taccatcagaggacacttggatt

SEQ ID NO: 597 - RNA, 23 nt, synthetic construct
  source 1..23: mol_type = other RNA
taggtgaaaacactgctttaggg

SEQ ID NO: 598 - RNA, 23 nt, synthetic construct
  source 1..23: mol_type = other RNA
tagaactttgaccatcagaggac

SEQ ID NO: 599 - RNA, 23 nt, synthetic construct
  source 1..23: mol_type = other RNA
tagaactttgaccatcagaggac

SEQ ID NO: 600 - RNA, 23 nt, synthetic construct
  source 1..23: mol_type = other RNA
tagaactttgaccatcagaggac

SEQ ID NO: 601 - RNA, 21 nt, synthetic construct
  source 1..21: mol_type = other RNA
ctaaagcagtgttttcaccta

SEQ ID NO: 602 - RNA, 23 nt, synthetic construct
  source 1..23: mol_type = other RNA
tagaactttgaccatcagaggac

SEQ ID NO: 603 - RNA, 21 nt, synthetic construct
  source 1..21: mol_type = other RNA
ctaaagcagtgttttcaccta

SEQ ID NO: 604 - RNA, 23 nt, synthetic construct
  source 1..23: mol_type = other RNA
taggtgaaaacactgctttaggg

SEQ ID NO: 605 - RNA, 21 nt, synthetic construct
  source 1..21: mol_type = other RNA
agcagtgttttcacctcatat

SEQ ID NO: 606 - RNA, 23 nt, synthetic construct
  source 1..23: mol_type = other RNA
atatgaggtgaaaacactgctgg

SEQ ID NO: 607 - RNA, 23 nt, synthetic construct
  source 1..23: mol_type = other RNA
tagaactttgaccatcagaggac

SEQ ID NO: 608 - RNA, 23 nt, synthetic construct
  source 1..23: mol_type = other RNA
tagaactttgaccatcagaggac

SEQ ID NO: 609 - RNA, 23 nt, synthetic construct
  source 1..23: mol_type = other RNA
tagaactttgaccatcagaggac

SEQ ID NO: 610 - RNA, 23 nt, synthetic construct
  source 1..23: mol_type = other RNA
tagaactttgaccatcagaggac

SEQ ID NO: 611 - RNA, 23 nt, synthetic construct
  source 1..23: mol_type = other RNA
tagaactttgaccatcagaggac

SEQ ID NO: 612 - RNA, 23 nt, synthetic construct
  source 1..23: mol_type = other RNA
tagaactttgaccatcagaggac

SEQ ID NO: 613 - RNA, 23 nt, synthetic construct
  source 1..23: mol_type = other RNA
tagaactttgaccatcagaggac

SEQ ID NO: 614 - RNA, 23 nt, synthetic construct
  source 1..23: mol_type = other RNA
tagaactttgaccatcagaggac

SEQ ID NO: 615 - RNA, 23 nt, synthetic construct
  source 1..23: mol_type = other RNA
tagaactttgaccatcagaggac

SEQ ID NO: 616 - RNA, 23 nt, synthetic construct
  source 1..23: mol_type = other RNA
tagaactttgaccatcagaggac

SEQ ID NO: 617 - RNA, 21 nt, synthetic construct
  source 1..21: mol_type = other RNA
agcagtgttttcacctcatat

SEQ ID NO: 618 - RNA, 23 nt, synthetic construct
  source 1..23: mol_type = other RNA
tagaactttgaccatcagaggac

SEQ ID NO: 619 - RNA, 23 nt, synthetic construct
  source 1..23: mol_type = other RNA
tagaactttgaccatcagaggac

SEQ ID NO: 620 - RNA, 23 nt, synthetic construct
  source 1..23: mol_type = other RNA
atatgaggtgaaaacactgctgg

SEQ ID NO: 621 - RNA, 23 nt, synthetic construct
  source 1..23: mol_type = other RNA
ttatgaggtgaaaacactgctgg

SEQ ID NO: 622 - RNA, 23 nt, synthetic construct
  source 1..23: mol_type = other RNA
tagaactttgaccatcagaggac

SEQ ID NO: 623 - RNA, 23 nt, synthetic construct
  source 1..23: mol_type = other RNA
tagaactttgaccatcagaggac

SEQ ID NO: 624 - RNA, 23 nt, synthetic construct
  source 1..23: mol_type = other RNA
tagaactttgaccatcagaggac

SEQ ID NO: 625 - RNA, 23 nt, synthetic construct
  source 1..23: mol_type = other RNA
tagaactttgaccatcagaggac

SEQ ID NO: 626 - RNA, 23 nt, synthetic construct
  source 1..23: mol_type = other RNA
tagaactttgaccatcagaggac

SEQ ID NO: 627 - RNA, 23 nt, synthetic construct
  source 1..23: mol_type = other RNA
tagaactttgaccatcagaggac

SEQ ID NO: 628 - RNA, 23 nt, synthetic construct
  source 1..23: mol_type = other RNA
atctagaactttgaccatcagag

SEQ ID NO: 629 - RNA, 23 nt, synthetic construct
  source 1..23: mol_type = other RNA
ttctagaactttgaccatcagag

SEQ ID NO: 630 - RNA, 23 nt, synthetic construct
  source 1..23: mol_type = other RNA
ttctagaactttgaccatcagag

SEQ ID NO: 631 - RNA, 23 nt, synthetic construct
  source 1..23: mol_type = other RNA
ttctagaactttgaccatcagag

SEQ ID NO: 632 - RNA, 23 nt, synthetic construct
  source 1..23: mol_type = other RNA
atctagaactttgaccatcagag

SEQ ID NO: 633 - RNA, 23 nt, synthetic construct
  source 1..23: mol_type = other RNA
atctagaactttgaccatcagag

SEQ ID NO: 634 - RNA, 23 nt, synthetic construct
  source 1..23: mol_type = other RNA
atctagaactttgaccatcagag

SEQ ID NO: 635 - RNA, 23 nt, synthetic construct
  source 1..23: mol_type = other RNA
atctagaactttgaccatcagag

SEQ ID NO: 636 - RNA, 23 nt, synthetic construct
  source 1..23: mol_type = other RNA
atctagaactttgaccatcagag

SEQ ID NO: 637 - RNA, 23 nt, synthetic construct
  source 1..23: mol_type = other RNA
atctagaactttgaccatcagag

SEQ ID NO: 638 - RNA, 23 nt, synthetic construct
  source 1..23: mol_type = other RNA
atctagaactttgaccatcagag

SEQ ID NO: 639 - RNA, 23 nt, synthetic construct
  source 1..23: mol_type = other RNA
atctagaactttgaccatcagag

SEQ ID NO: 640 - RNA, 23 nt, synthetic construct
  source 1..23: mol_type = other RNA
atctagaactttgaccatcagag

SEQ ID NO: 641 - RNA, 21 nt, synthetic construct
  source 1..21: mol_type = other RNA
aggcagagacaataaaacatt

SEQ ID NO: 642 - RNA, 23 nt, synthetic construct
  source 1..23: mol_type = other RNA
atctagaactttgaccatcagag

SEQ ID NO: 643 - RNA, 23 nt, synthetic construct
  source 1..23: mol_type = other RNA
atctagaactttgaccatcagag

SEQ ID NO: 644 - RNA, 23 nt, synthetic construct
  source 1..23: mol_type = other RNA
aatgttttattgtctctgcctgg

SEQ ID NO: 645 - RNA, 23 nt, synthetic construct
  source 1..23: mol_type = other RNA
atctagaactttgaccatcagag

SEQ ID NO: 646 - RNA, 23 nt, synthetic construct
  source 1..23: mol_type = other RNA
atctagaactttgaccatcagag

SEQ ID NO: 647 - RNA, 23 nt, synthetic construct
  source 1..23: mol_type = other RNA
atctagaactttgaccatcagag

SEQ ID NO: 648 - RNA, 23 nt, synthetic construct
  source 1..23: mol_type = other RNA
atctagaactttgaccatcagag

SEQ ID NO: 649 - RNA, 23 nt, synthetic construct
  source 1..23: mol_type = other RNA
atctagaactttgaccatcagag

SEQ ID NO: 650 - RNA, 23 nt, synthetic construct
  source 1..23: mol_type = other RNA
atctagaactttgaccatcagag

SEQ ID NO: 651 - RNA, 23 nt, synthetic construct
  source 1..23: mol_type = other RNA
atctagaactttgaccatcagag

SEQ ID NO: 652 - RNA, 23 nt, synthetic construct
  source 1..23: mol_type = other RNA
tctatttccactttgtatatccc

SEQ ID NO: 653 - RNA, 21 nt, synthetic construct
  source 1..21: mol_type = other RNA
aggcagagacaataaaacatt

SEQ ID NO: 654 - RNA, 23 nt, synthetic construct
  source 1..23: mol_type = other RNA
tctatttccactttgtatatccc

SEQ ID NO: 655 - RNA, 23 nt, synthetic construct
  source 1..23: mol_type = other RNA
aatgttttattgtctctgcctgg

SEQ ID NO: 656 - RNA, 23 nt, synthetic construct
  source 1..23: mol_type = other RNA
tctatttccactttgtatatccc

SEQ ID NO: 657 - RNA, 23 nt, synthetic construct
  source 1..23: mol_type = other RNA
tctatttccactttgtatatccc

SEQ ID NO: 658 - RNA, 23 nt, synthetic construct
  source 1..23: mol_type = other RNA
tctatttccactttgtatatccc

SEQ ID NO: 659 - RNA, 23 nt, synthetic construct
  source 1..23: mol_type = other RNA
tctatttccactttgtatatccc

SEQ ID NO: 660 - RNA, 23 nt, synthetic construct
  source 1..23: mol_type = other RNA
tctatttccactttgtatatccc

SEQ ID NO: 661 - RNA, 23 nt, synthetic construct
  source 1..23: mol_type = other RNA
tctatttccactttgtatatccc

SEQ ID NO: 662 - RNA, 23 nt, synthetic construct
  source 1..23: mol_type = other RNA
tctatttccactttgtatatccc

SEQ ID NO: 663 - RNA, 23 nt, synthetic construct
  source 1..23: mol_type = other RNA
tctatttccactttgtatatccc

SEQ ID NO: 664 - RNA, 23 nt, synthetic construct
  source 1..23: mol_type = other RNA
tctatttccactttgtatatccc

SEQ ID NO: 665 - RNA, 23 nt, synthetic construct
  source 1..23: mol_type = other RNA
tctatttccactttgtatatccc

SEQ ID NO: 666 - RNA, 23 nt, synthetic construct
  source 1..23: mol_type = other RNA
tctatttccactttgtatatccc

SEQ ID NO: 667 - RNA, 23 nt, synthetic construct
  source 1..23: mol_type = other RNA
tctatttccactttgtatatccc

SEQ ID NO: 668 - RNA, 23 nt, synthetic construct
  source 1..23: mol_type = other RNA
tctatttccactttgtatatccc

SEQ ID NO: 669 - RNA, 23 nt, synthetic construct
  source 1..23: mol_type = other RNA
tctatttccactttgtatatccc

SEQ ID NO: 670 - RNA, 23 nt, synthetic construct
  source 1..23: mol_type = other RNA
tctatttccactttgtatatccc

SEQ ID NO: 671 - RNA, 23 nt, synthetic construct
  source 1..23: mol_type = other RNA
tctatttccactttgtatatccc

SEQ ID NO: 672 - RNA, 23 nt, synthetic construct
  source 1..23: mol_type = other RNA
tctatttccactttgtatatccc

SEQ ID NO: 673 - RNA, 23 nt, synthetic construct
  source 1..23: mol_type = other RNA
tctatttccactttgtatatccc

SEQ ID NO: 674 - RNA, 23 nt, synthetic construct
  source 1..23: mol_type = other RNA
tctatttccactttgtatatccc

SEQ ID NO: 675 - RNA, 23 nt, synthetic construct
  source 1..23: mol_type = other RNA
tctatttccactttgtatatccc

SEQ ID NO: 676 - RNA, 23 nt, synthetic construct
  source 1..23: mol_type = other RNA
taagatttggtgtctatttccac

SEQ ID NO: 677 - RNA, 23 nt, synthetic construct
  source 1..23: mol_type = other RNA
taagatttggtgtctatttccac

SEQ ID NO: 678 - RNA, 23 nt, synthetic construct
  source 1..23: mol_type = other RNA
taagatttggtgtctatttccac

SEQ ID NO: 679 - RNA, 23 nt, synthetic construct
  source 1..23: mol_type = other RNA
taagatttggtgtctatttccac

SEQ ID NO: 680 - RNA, 23 nt, synthetic construct
  source 1..23: mol_type = other RNA
taagatttggtgtctatttccac

SEQ ID NO: 681 - RNA, 23 nt, synthetic construct
  source 1..23: mol_type = other RNA
taagatttggtgtctatttccac

SEQ ID NO: 682 - RNA, 23 nt, synthetic construct
  source 1..23: mol_type = other RNA
taagatttggtgtctatttccac

SEQ ID NO: 683 - RNA, 23 nt, synthetic construct
  source 1..23: mol_type = other RNA
taagatttggtgtctatttccac

SEQ ID NO: 684 - RNA, 23 nt, synthetic construct
  source 1..23: mol_type = other RNA
taagatttggtgtctatttccac

SEQ ID NO: 685 - RNA, 23 nt, synthetic construct
  source 1..23: mol_type = other RNA
taagatttggtgtctatttccac

SEQ ID NO: 686 - RNA, 23 nt, synthetic construct
  source 1..23: mol_type = other RNA
taagatttggtgtctatttccac

SEQ ID NO: 687 - RNA, 23 nt, synthetic construct
  source 1..23: mol_type = other RNA
taagatttggtgtctatttccac

SEQ ID NO: 688 - RNA, 23 nt, synthetic construct
  source 1..23: mol_type = other RNA
taagatttggtgtctatttccac

SEQ ID NO: 689 - RNA, 23 nt, synthetic construct
  source 1..23: mol_type = other RNA
taagatttggtgtctatttccac

SEQ ID NO: 690 - RNA, 23 nt, synthetic construct
  source 1..23: mol_type = other RNA
taagatttggtgtctatttccac

SEQ ID NO: 691 - RNA, 23 nt, synthetic construct
  source 1..23: mol_type = other RNA
taagatttggtgtctatttccac

SEQ ID NO: 692 - RNA, 23 nt, synthetic construct
  source 1..23: mol_type = other RNA
taagatttggtgtctatttccac

SEQ ID NO: 693 - RNA, 23 nt, synthetic construct
  source 1..23: mol_type = other RNA
taagatttggtgtctatttccac

SEQ ID NO: 694 - RNA, 23 nt, synthetic construct
  source 1..23: mol_type = other RNA
taagatttggtgtctatttccac

SEQ ID NO: 695 - RNA, 23 nt, synthetic construct
  source 1..23: mol_type = other RNA
taagatttggtgtctatttccac

SEQ ID NO: 696 - RNA, 23 nt, synthetic construct
  source 1..23: mol_type = other RNA
taagatttggtgtctatttccac

SEQ ID NO: 697 - RNA, 23 nt, synthetic construct
  source 1..23: mol_type = other RNA
taagatttggtgtctatttccac

SEQ ID NO: 698 - RNA, 23 nt, synthetic construct
  source 1..23: mol_type = other RNA
ttgtgaataccacctctgcatgc

SEQ ID NO: 699 - RNA, 23 nt, synthetic construct
  source 1..23: mol_type = other RNA
ttgtgaataccacctctgcatgc

SEQ ID NO: 700 - RNA, 23 nt, synthetic construct
  source 1..23: mol_type = other RNA
ttgtgaataccacctctgcatgc

SEQ ID NO: 701 - RNA, 23 nt, synthetic construct
  source 1..23: mol_type = other RNA
ttgtgaataccacctctgcatgc

SEQ ID NO: 702 - RNA, 23 nt, synthetic construct
  source 1..23: mol_type = other RNA
ttgtgaataccacctctgcatgc

SEQ ID NO: 703 - RNA, 23 nt, synthetic construct
  source 1..23: mol_type = other RNA
ttgtgaataccacctctgcatgc

SEQ ID NO: 704 - RNA, 23 nt, synthetic construct
  source 1..23: mol_type = other RNA
ttgtgaataccacctctgcatgc

SEQ ID NO: 705 - RNA, 23 nt, synthetic construct
  source 1..23: mol_type = other RNA
ttgtgaataccacctctgcatgc

SEQ ID NO: 706 - RNA, 23 nt, synthetic construct
  source 1..23: mol_type = other RNA
ttgtgaataccacctctgcatgc

SEQ ID NO: 707 - RNA, 23 nt, synthetic construct
  source 1..23: mol_type = other RNA
ttgtgaataccacctctgcatgc

SEQ ID NO: 708 - RNA, 23 nt, synthetic construct
  source 1..23: mol_type = other RNA
ttgtgaataccacctctgcatgc

SEQ ID NO: 709 - RNA, 23 nt, synthetic construct
  source 1..23: mol_type = other RNA
ttgtgaataccacctctgcatgc

SEQ ID NO: 710 - RNA, 23 nt, synthetic construct
  source 1..23: mol_type = other RNA
ttgtgaataccacctctgcatgc

SEQ ID NO: 711 - RNA, 23 nt, synthetic construct
  source 1..23: mol_type = other RNA
ttgtgaataccacctctgcatgc

SEQ ID NO: 712 - RNA, 23 nt, synthetic construct
  source 1..23: mol_type = other RNA
ttgtgaataccacctctgcatgc

SEQ ID NO: 713 - RNA, 23 nt, synthetic construct
  source 1..23: mol_type = other RNA
ttgtgaataccacctctgcatgc

SEQ ID NO: 714 - RNA, 23 nt, synthetic construct
  source 1..23: mol_type = other RNA
tttcacaggaatgttttattgtc

SEQ ID NO: 715 - RNA, 23 nt, synthetic construct
  source 1..23: mol_type = other RNA
ttgtgaataccacctctgcatgc

SEQ ID NO: 716 - RNA, 23 nt, synthetic construct
  source 1..23: mol_type = other RNA
ttgtgaataccacctctgcatgc

SEQ ID NO: 717 - RNA, 23 nt, synthetic construct
  source 1..23: mol_type = other RNA
ttgtgaataccacctctgcatgc

SEQ ID NO: 718 - RNA, 23 nt, synthetic construct
  source 1..23: mol_type = other RNA
ttgtgaataccacctctgcatgc

SEQ ID NO: 719 - RNA, 23 nt, synthetic construct
  source 1..23: mol_type = other RNA
ttgtgaataccacctctgcatgc

SEQ ID NO: 720 - RNA, 23 nt, synthetic construct
  source 1..23: mol_type = other RNA
taggagtaggggctcagcagggc

SEQ ID NO: 721 - RNA, 23 nt, synthetic construct
  source 1..23: mol_type = other RNA
taggagtaggggctcagcagggc

SEQ ID NO: 722 - RNA, 23 nt, synthetic construct
  source 1..23: mol_type = other RNA
taggagtaggggctcagcagggc

SEQ ID NO: 723 - RNA, 23 nt, synthetic construct
  source 1..23: mol_type = other RNA
ttgtgaataccacctctgcatgc

SEQ ID NO: 724 - RNA, 23 nt, synthetic construct
  source 1..23: mol_type = other RNA
taggagtaggggctcagcagggc

SEQ ID NO: 725 - RNA, 23 nt, synthetic construct
  source 1..23: mol_type = other RNA
taggagtaggggctcagcagggc

SEQ ID NO: 726 - RNA, 23 nt, synthetic construct
  source 1..23: mol_type = other RNA
taggagtaggggctcagcagggc

SEQ ID NO: 727 - RNA, 23 nt, synthetic construct
  source 1..23: mol_type = other RNA
taggagtaggggctcagcagggc

SEQ ID NO: 728 - RNA, 23 nt, synthetic construct
  source 1..23: mol_type = other RNA
taggagtaggggctcagcagggc

SEQ ID NO: 729 - RNA, 23 nt, synthetic construct
  source 1..23: mol_type = other RNA
taggagtaggggctcagcagggc

SEQ ID NO: 730 - RNA, 23 nt, synthetic construct
  source 1..23: mol_type = other RNA
taggagtaggggctcagcagggc

SEQ ID NO: 731 - RNA, 23 nt, synthetic construct
  source 1..23: mol_type = other RNA
taggagtaggggctcagcagggc

SEQ ID NO: 732 - RNA, 23 nt, synthetic construct
  source 1..23: mol_type = other RNA
taggagtaggggctcagcagggc

SEQ ID NO: 733 - RNA, 23 nt, synthetic construct
  source 1..23: mol_type = other RNA
taggagtaggggctcagcagggc

SEQ ID NO: 734 - RNA, 23 nt, synthetic construct
  source 1..23: mol_type = other RNA
taggagtaggggctcagcagggc

SEQ ID NO: 735 - RNA, 23 nt, synthetic construct
  source 1..23: mol_type = other RNA
taggagtaggggctcagcagggc

SEQ ID NO: 736 - RNA, 23 nt, synthetic construct
  source 1..23: mol_type = other RNA
taggagtaggggctcagcagggc

SEQ ID NO: 737 - RNA, 23 nt, synthetic construct
  source 1..23: mol_type = other RNA
taggagtaggggctcagcagggc

SEQ ID NO: 738 - RNA, 23 nt, synthetic construct
  source 1..23: mol_type = other RNA
taggagtaggggctcagcagggc

SEQ ID NO: 739 - RNA, 23 nt, synthetic construct
  source 1..23: mol_type = other RNA
taggagtaggggctcagcagggc

SEQ ID NO: 740 - RNA, 23 nt, synthetic construct
  source 1..23: mol_type = other RNA
taggagtaggggctcagcagggc

SEQ ID NO: 741 - RNA, 23 nt, synthetic construct
  source 1..23: mol_type = other RNA
taggagtaggggctcagcagggc

SEQ ID NO: 742 - RNA, 23 nt, synthetic construct
  source 1..23: mol_type = other RNA
taggagtaggggctcagcagggc

SEQ ID NO: 743 - RNA, 23 nt, synthetic construct
  source 1..23: mol_type = other RNA
taggtgaaaacactgctttaggg

SEQ ID NO: 744 - RNA, 21 nt, synthetic construct
  source 1..21: mol_type = other RNA
agcagtgttttcacctcataa

SEQ ID NO: 745 - RNA, 23 nt, synthetic construct
  source 1..23: mol_type = other RNA
taggtgaaaacactgctttaggg

SEQ ID NO: 746 - RNA, 23 nt, synthetic construct
  source 1..23: mol_type = other RNA
taggtgaaaacactgctttaggg

SEQ ID NO: 747 - RNA, 23 nt, synthetic construct
  source 1..23: mol_type = other RNA
taggtgaaaacactgctttaggg

SEQ ID NO: 748 - RNA, 23 nt, synthetic construct
  source 1..23: mol_type = other RNA
tttcacaggaatgttttattgtc

SEQ ID NO: 749 - RNA, 23 nt, synthetic construct
  source 1..23: mol_type = other RNA
taggtgaaaacactgctttaggg

SEQ ID NO: 750 - RNA, 23 nt, synthetic construct
  source 1..23: mol_type = other RNA
taggtgaaaacactgctttaggg

SEQ ID NO: 751 - RNA, 21 nt, synthetic construct
  source 1..21: mol_type = other RNA
agcagtgttttcacctcatat

SEQ ID NO: 752 - RNA, 21 nt, synthetic construct
  source 1..21: mol_type = other RNA
agcagtgttttcacctcatat

SEQ ID NO: 753 - RNA, 21 nt, synthetic construct
  source 1..21: mol_type = other RNA
agcagtgttttcacctcataa

SEQ ID NO: 754 - RNA, 21 nt, synthetic construct
  source 1..21: mol_type = other RNA
agcagtgttttcacctcataa

SEQ ID NO: 755 - RNA, 21 nt, synthetic construct
  source 1..21: mol_type = other RNA
ctaaagcagtgttttcaccta

SEQ ID NO: 756 - RNA, 21 nt, synthetic construct
  source 1..21: mol_type = other RNA
ctaaagcagtgttttcaccta

SEQ ID NO: 757 - RNA, 21 nt, synthetic construct
  source 1..21: mol_type = other RNA
aggcagagacaataaaacatt

SEQ ID NO: 758 - RNA, 21 nt, synthetic construct
  source 1..21: mol_type = other RNA
aggcagagacaataaaacatt

SEQ ID NO: 759 - RNA, 21 nt, synthetic construct
  source 1..21: mol_type = other RNA
aggcagagacaataaaacatt

SEQ ID NO: 760 - RNA, 21 nt, synthetic construct
  source 1..21: mol_type = other RNA
agcagtgttttcacctcatat

SEQ ID NO: 761 - RNA, 21 nt, synthetic construct
  source 1..21: mol_type = other RNA
agcagtgttttcacctcataa

SEQ ID NO: 762 - RNA, 21 nt, synthetic construct
  source 1..21: mol_type = other RNA
ctaaagcagtgttttcaccta

SEQ ID NO: 763 - RNA, 23 nt, synthetic construct
  source 1..23: mol_type = other RNA
taggtgaaaacactgctttaggg

SEQ ID NO: 764 - RNA, 23 nt, synthetic construct
  source 1..23: mol_type = other RNA
taggtgaaaacactgctttaggg

SEQ ID NO: 765 - RNA, 23 nt, synthetic construct
  source 1..23: mol_type = other RNA
taggtgaaaacactgctttaggg

SEQ ID NO: 766 - RNA, 23 nt, synthetic construct
  source 1..23: mol_type = other RNA
taggtgaaaacactgctttaggg

SEQ ID NO: 767 - RNA, 23 nt, synthetic construct
  source 1..23: mol_type = other RNA
taggtgaaaacactgctttaggg

SEQ ID NO: 768 - RNA, 23 nt, synthetic construct
  source 1..23: mol_type = other RNA
taggtgaaaacactgctttaggg

SEQ ID NO: 769 - RNA, 23 nt, synthetic construct
  source 1..23: mol_type = other RNA
taggtgaaaacactgctttaggg

SEQ ID NO: 770 - RNA, 23 nt, synthetic construct
  source 1..23: mol_type = other RNA
taggtgaaaacactgctttaggg

SEQ ID NO: 771 - RNA, 23 nt, synthetic construct
  source 1..23: mol_type = other RNA
taggtgaaaacactgctttaggg

SEQ ID NO: 772 - RNA, 23 nt, synthetic construct
  source 1..23: mol_type = other RNA
taggtgaaaacactgctttaggg

SEQ ID NO: 773 - RNA, 23 nt, synthetic construct
  source 1..23: mol_type = other RNA
taggtgaaaacactgctttaggg

SEQ ID NO: 774 - RNA, 23 nt, synthetic construct
  source 1..23: mol_type = other RNA
ttatgaggtgaaaacactgctgg

SEQ ID NO: 775 - RNA, 23 nt, synthetic construct
  source 1..23: mol_type = other RNA
atatgaggtgaaaacactgctgg

SEQ ID NO: 776 - RNA, 23 nt, synthetic construct
  source 1..23: mol_type = other RNA
atatgaggtgaaaacactgctgg

SEQ ID NO: 777 - RNA, 23 nt, synthetic construct
  source 1..23: mol_type = other RNA
atatgaggtgaaaacactgctgg

SEQ ID NO: 778 - RNA, 23 nt, synthetic construct
  source 1..23: mol_type = other RNA
ttatgaggtgaaaacactgctgg

SEQ ID NO: 779 - RNA, 23 nt, synthetic construct
  source 1..23: mol_type = other RNA
atatgaggtgaaaacactgctgg

SEQ ID NO: 780 - RNA, 23 nt, synthetic construct
  source 1..23: mol_type = other RNA
atatgaggtgaaaacactgctgg

SEQ ID NO: 781 - RNA, 23 nt, synthetic construct
  source 1..23: mol_type = other RNA
atatgaggtgaaaacactgctgg

SEQ ID NO: 782 - RNA, 23 nt, synthetic construct
  source 1..23: mol_type = other RNA
atatgaggtgaaaacactgctgg

SEQ ID NO: 783 - RNA, 23 nt, synthetic construct
  source 1..23: mol_type = other RNA
atatgaggtgaaaacactgctgg

SEQ ID NO: 784 - RNA, 23 nt, synthetic construct
  source 1..23: mol_type = other RNA
atatgaggtgaaaacactgctgg

SEQ ID NO: 785 - RNA, 23 nt, synthetic construct
  source 1..23: mol_type = other RNA
atatgaggtgaaaacactgctgt

SEQ ID NO: 786 - RNA, 23 nt, synthetic construct
  source 1..23: mol_type = other RNA
atatgaggtgaaaacactgctgg

SEQ ID NO: 787 - RNA, 23 nt, synthetic construct
  source 1..23: mol_type = other RNA
atatgaggtgaaaacactgcttt

SEQ ID NO: 788 - RNA, 23 nt, synthetic construct
  source 1..23: mol_type = other RNA
atatgaggtgaaaacactgctgg

SEQ ID NO: 789 - RNA, 23 nt, synthetic construct
  source 1..23: mol_type = other RNA
atatgaggtgaaaacactgctgg

SEQ ID NO: 790 - RNA, 23 nt, synthetic construct
  source 1..23: mol_type = other RNA
atatgaggtgaaaacactgctgg

SEQ ID NO: 791 - RNA, 23 nt, synthetic construct
  source 1..23: mol_type = other RNA
atatgaggtgaaaacactgctgg

SEQ ID NO: 792 - RNA, 23 nt, synthetic construct
  source 1..23: mol_type = other RNA
atatgaggtgaaaacactgctgg

SEQ ID NO: 793 - RNA, 23 nt, synthetic construct
  source 1..23: mol_type = other RNA
atatgaggtgaaaacactgctgg

SEQ ID NO: 794 - RNA, 23 nt, synthetic construct
  source 1..23: mol_type = other RNA
ttttattgtctctgcctggactt

SEQ ID NO: 795 - RNA, 23 nt, synthetic construct
  source 1..23: mol_type = other RNA
ttttattgtctctgcctggactt

SEQ ID NO: 796 - RNA, 23 nt, synthetic construct
  source 1..23: mol_type = other RNA
ttttattgtctctgcctggactt

SEQ ID NO: 797 - RNA, 23 nt, synthetic construct
  source 1..23: mol_type = other RNA
ttttattgtctctgcctggactt

SEQ ID NO: 798 - RNA, 23 nt, synthetic construct
  source 1..23: mol_type = other RNA
ttttattgtctctgcctggactt

SEQ ID NO: 799 - RNA, 23 nt, synthetic construct
  source 1..23: mol_type = other RNA
ttttattgtctctgcctggactt

SEQ ID NO: 800 - RNA, 23 nt, synthetic construct
  source 1..23: mol_type = other RNA
ttttattgtctctgcctggactt

SEQ ID NO: 801 - RNA, 23 nt, synthetic construct
  source 1..23: mol_type = other RNA
ttttattgtctctgcctggactt

SEQ ID NO: 802 - RNA, 23 nt, synthetic construct
  source 1..23: mol_type = other RNA
ttttattgtctctgcctggactt

SEQ ID NO: 803 - RNA, 23 nt, synthetic construct
  source 1..23: mol_type = other RNA
ttttattgtctctgcctggactt

SEQ ID NO: 804 - RNA, 23 nt, synthetic construct
  source 1..23: mol_type = other RNA
ttttattgtctctgcctggactt

SEQ ID NO: 805 - RNA, 23 nt, synthetic construct
  source 1..23: mol_type = other RNA
ttttattgtctctgcctggactt

SEQ ID NO: 806 - RNA, 23 nt, synthetic construct
  source 1..23: mol_type = other RNA
ttttattgtctctgcctggactt

SEQ ID NO: 807 - RNA, 23 nt, synthetic construct
  source 1..23: mol_type = other RNA
ttttattgtctctgcctggactt

SEQ ID NO: 808 - RNA, 23 nt, synthetic construct
  source 1..23: mol_type = other RNA
ttttattgtctctgcctggactt

SEQ ID NO: 809 - RNA, 23 nt, synthetic construct
  source 1..23: mol_type = other RNA
ttttattgtctctgcctggactt

SEQ ID NO: 810 - RNA, 23 nt, synthetic construct
  source 1..23: mol_type = other RNA
ttttattgtctctgcctggactt

SEQ ID NO: 811 - RNA, 23 nt, synthetic construct
  source 1..23: mol_type = other RNA
ttttattgtctctgcctggactt

SEQ ID NO: 812 - RNA, 23 nt, synthetic construct
  source 1..23: mol_type = other RNA
ttttattgtctctgcctggactt

SEQ ID NO: 813 - RNA, 23 nt, synthetic construct
  source 1..23: mol_type = other RNA
ttttattgtctctgcctggactt

SEQ ID NO: 814 - RNA, 23 nt, synthetic construct
  source 1..23: mol_type = other RNA
aatgttttattgtctctgcctgg

SEQ ID NO: 815 - RNA, 23 nt, synthetic construct
  source 1..23: mol_type = other RNA
aatgttttattgtctctgcctgg

SEQ ID NO: 816 - RNA, 23 nt, synthetic construct
  source 1..23: mol_type = other RNA
aatgttttattgtctctgcctgg

SEQ ID NO: 817 - RNA, 23 nt, synthetic construct
  source 1..23: mol_type = other RNA
aatgttttattgtctctgcctgg

SEQ ID NO: 818 - RNA, 23 nt, synthetic construct
  source 1..23: mol_type = other RNA
aatgttttattgtctctgcctgg

SEQ ID NO: 819 - RNA, 23 nt, synthetic construct
  source 1..23: mol_type = other RNA
aatgttttattgtctctgcctgg

SEQ ID NO: 820 - RNA, 23 nt, synthetic construct
  source 1..23: mol_type = other RNA
aatgttttattgtctctgcctgg

SEQ ID NO: 821 - RNA, 23 nt, synthetic construct
  source 1..23: mol_type = other RNA
tatgttttattgtctctgcctgg

SEQ ID NO: 822 - RNA, 23 nt, synthetic construct
  source 1..23: mol_type = other RNA
tatgttttattgtctctgcctgg

SEQ ID NO: 823 - RNA, 23 nt, synthetic construct
  source 1..23: mol_type = other RNA
aatgttttattgtctctgcctgg

SEQ ID NO: 824 - RNA, 23 nt, synthetic construct
  source 1..23: mol_type = other RNA
aatgttttattgtctctgcctgg

SEQ ID NO: 825 - RNA, 23 nt, synthetic construct
  source 1..23: mol_type = other RNA
tatgttttattgtctctgcctgg

SEQ ID NO: 826 - RNA, 23 nt, synthetic construct
  source 1..23: mol_type = other RNA
aatgttttattgtctctgcctgg

SEQ ID NO: 827 - RNA, 23 nt, synthetic construct
  source 1..23: mol_type = other RNA
aatgttttattgtctctgcctgg

SEQ ID NO: 828 - RNA, 23 nt, synthetic construct
  source 1..23: mol_type = other RNA
aatgttttattgtctctgcctgg

SEQ ID NO: 829 - RNA, 23 nt, synthetic construct
  source 1..23: mol_type = other RNA
aatgttttattgtctctgcctgg

SEQ ID NO: 830 - RNA, 23 nt, synthetic construct
  source 1..23: mol_type = other RNA
aatgttttattgtctctgcctgg

SEQ ID NO: 831 - RNA, 23 nt, synthetic construct
  source 1..23: mol_type = other RNA
aatgttttattgtctctgcctgg

SEQ ID NO: 832 - RNA, 23 nt, synthetic construct
  source 1..23: mol_type = other RNA
aatgttttattgtctctgcctgg

SEQ ID NO: 833 - RNA, 23 nt, synthetic construct
  source 1..23: mol_type = other RNA
aatgttttattgtctctgcctgg

SEQ ID NO: 834 - RNA, 23 nt, synthetic construct
  source 1..23: mol_type = other RNA
taggaatgttttattgtctctgc

SEQ ID NO: 835 - RNA, 23 nt, synthetic construct
  source 1..23: mol_type = other RNA
taggaatgttttattgtctctgc

SEQ ID NO: 836 - RNA, 23 nt, synthetic construct
  source 1..23: mol_type = other RNA
taggaatgttttattgtctctgc

SEQ ID NO: 837 - RNA, 23 nt, synthetic construct
  source 1..23: mol_type = other RNA
taggaatgttttattgtctctgc

SEQ ID NO: 838 - RNA, 23 nt, synthetic construct
  source 1..23: mol_type = other RNA
taggaatgttttattgtctctgc

SEQ ID NO: 839 - RNA, 23 nt, synthetic construct
  source 1..23: mol_type = other RNA
taggaatgttttattgtctctgc

SEQ ID NO: 840 - RNA, 23 nt, synthetic construct
  source 1..23: mol_type = other RNA
taggaatgttttattgtctctgc

SEQ ID NO: 841 - RNA, 23 nt, synthetic construct
  source 1..23: mol_type = other RNA
taggaatgttttattgtctctgc

SEQ ID NO: 842 - RNA, 23 nt, synthetic construct
  source 1..23: mol_type = other RNA
taggaatgttttattgtctctgc

SEQ ID NO: 843 - RNA, 23 nt, synthetic construct
  source 1..23: mol_type = other RNA
taggaatgttttattgtctctgc

SEQ ID NO: 844 - RNA, 23 nt, synthetic construct
  source 1..23: mol_type = other RNA
taggaatgttttattgtctctgc

SEQ ID NO: 845 - RNA, 23 nt, synthetic construct
  source 1..23: mol_type = other RNA
taggaatgttttattgtctctgc

SEQ ID NO: 846 - RNA, 23 nt, synthetic construct
  source 1..23: mol_type = other RNA
taggaatgttttattgtctctgc

SEQ ID NO: 847 - RNA, 23 nt, synthetic construct
  source 1..23: mol_type = other RNA
taggaatgttttattgtctctgc

SEQ ID NO: 848 - RNA, 23 nt, synthetic construct
  source 1..23: mol_type = other RNA
taggaatgttttattgtctctgc

SEQ ID NO: 849 - RNA, 23 nt, synthetic construct
  source 1..23: mol_type = other RNA
taggaatgttttattgtctctgc

SEQ ID NO: 850 - RNA, 23 nt, synthetic construct
  source 1..23: mol_type = other RNA
taggaatgttttattgtctctgc

SEQ ID NO: 851 - RNA, 23 nt, synthetic construct
  source 1..23: mol_type = other RNA
taggaatgttttattgtctctgc

SEQ ID NO: 852 - RNA, 23 nt, synthetic construct
  source 1..23: mol_type = other RNA
taggaatgttttattgtctctgc

SEQ ID NO: 853 - RNA, 23 nt, synthetic construct
  source 1..23: mol_type = other RNA
taggaatgttttattgtctctgc

SEQ ID NO: 854 - RNA, 23 nt, synthetic construct
  source 1..23: mol_type = other RNA
taggaatgttttattgtctctgc

SEQ ID NO: 855 - RNA, 23 nt, synthetic construct
  source 1..23: mol_type = other RNA
taggaatgttttattgtctctgc

SEQ ID NO: 856 - RNA, 23 nt, synthetic construct
  source 1..23: mol_type = other RNA
tttcacaggaatgttttattgtc

SEQ ID NO: 857 - RNA, 23 nt, synthetic construct
  source 1..23: mol_type = other RNA
tttcacaggaatgttttattgtc

SEQ ID NO: 858 - RNA, 23 nt, synthetic construct
  source 1..23: mol_type = other RNA
tttcacaggaatgttttattgtc

SEQ ID NO: 859 - RNA, 23 nt, synthetic construct
  source 1..23: mol_type = other RNA
tttcacaggaatgttttattgtc

SEQ ID NO: 860 - RNA, 23 nt, synthetic construct
  source 1..23: mol_type = other RNA
tttcacaggaatgttttattgtc

SEQ ID NO: 861 - RNA, 23 nt, synthetic construct
  source 1..23: mol_type = other RNA
tttcacaggaatgttttattgtc

SEQ ID NO: 862 - RNA, 23 nt, synthetic construct
  source 1..23: mol_type = other RNA
tttcacaggaatgttttattgtc

SEQ ID NO: 863 - RNA, 23 nt, synthetic construct
  source 1..23: mol_type = other RNA
tttcacaggaatgttttattgtc

SEQ ID NO: 864 - RNA, 23 nt, synthetic construct
  source 1..23: mol_type = other RNA
tttcacaggaatgttttattgtc

SEQ ID NO: 865 - RNA, 23 nt, synthetic construct
  source 1..23: mol_type = other RNA
tttcacaggaatgttttattgtc

SEQ ID NO: 866 - RNA, 23 nt, synthetic construct
  source 1..23: mol_type = other RNA
tttcacaggaatgttttattgtc

SEQ ID NO: 867 - RNA, 23 nt, synthetic construct
  source 1..23: mol_type = other RNA
tttcacaggaatgttttattgtc

SEQ ID NO: 868 - RNA, 23 nt, synthetic construct
  source 1..23: mol_type = other RNA
tttcacaggaatgttttattgtc

SEQ ID NO: 869 - RNA, 23 nt, synthetic construct
  source 1..23: mol_type = other RNA
tttcacaggaatgttttattgtc

SEQ ID NO: 870 - RNA, 23 nt, synthetic construct
  source 1..23: mol_type = other RNA
tttcacaggaatgttttattgtc

SEQ ID NO: 871 - RNA, 23 nt, synthetic construct
  source 1..23: mol_type = other RNA
tttcacaggaatgttttattgtc

SEQ ID NO: 872 - RNA, 23 nt, synthetic construct
  source 1..23: mol_type = other RNA
tttcacaggaatgttttattgtc

SEQ ID NO: 873 - RNA, 23 nt, synthetic construct
  source 1..23: mol_type = other RNA
tttcacaggaatgttttattgtc

SEQ ID NO: 874 - RNA, 23 nt, synthetic construct
  source 1..23: mol_type = other RNA
tttcacaggaatgttttattgtc

SEQ ID NO: 875 - RNA, 23 nt, synthetic construct
  source 1..23: mol_type = other RNA
tttcacaggaatgttttattgtc

SEQ ID NO: 876 - RNA, 21 nt, synthetic construct
  source 1..21: mol_type = other RNA
tgggatttcatgtaaccaaga

SEQ ID NO: 877 - RNA, 23 nt, synthetic construct
  source 1..23: mol_type = other RNA
tcttggttacatgaaatcccatc

SEQ ID NO: 878 - RNA, 23 nt, synthetic construct
  source 1..23: mol_type = other RNA
taggtgaaaacactgctttaggg

SEQ ID NO: 879 - RNA, 23 nt, synthetic construct
  source 1..23: mol_type = other RNA
taggtgaaaacactgctttaggg

SEQ ID NO: 880 - RNA, 23 nt, synthetic construct
  source 1..23: mol_type = other RNA
taggtgaaaacactgctttaggg

SEQ ID NO: 881 - RNA, 23 nt, synthetic construct
  source 1..23: mol_type = other RNA
atatgaggtgaaaacactgctgg

SEQ ID NO: 882 - RNA, 23 nt, synthetic construct
  source 1..23: mol_type = other RNA
ttttattgtctctgcctggactt

SEQ ID NO: 883 - RNA, 23 nt, synthetic construct
  source 1..23: mol_type = other RNA
ttttattgtctctgcctggactt

SEQ ID NO: 884 - RNA, 616 nt, Homo sapiens
  source 1..616: mol_type = mRNA
acagaagtccactcattcttggcaggatggcttctcatcgtctgctcctcctctgccttgctggactggtatttgtgtctgaggctggccctacgggcaccggtgaatccaagtgtcctctgatggtcaaagttctagatgctgtccgaggcagtcctgccatcaatgtggccgtgcatgtgttcagaaaggctgctgatgacacctgggagccatttgcctctgggaaaaccagtgagtctggagagctgcatgggctcacaactgaggaggaatttgtagaagggatatacaaagtggaaatagacaccaaatcttactggaaggcacttggcatctccccattccatgagcatgcagaggtggtattcacagccaacgactccggcccccgccgctacaccattgccgccctgctgagcccctactcctattccaccacggctgtcgtcaccaatcccaaggaatgagggacttctcctccagtggacctgaaggacgagggatgggatttcatgtaaccaagagtattccatttttactaaagcagtgttttcacctcatatgctatgttagaagtccaggcagagacaataaaacattcctgtgaaaggca

SEQ ID NO: 885 - DNA, 19 bp, synthetic construct
  source 1..19: mol_type = other DNA
cccctactcctattccacc

SEQ ID NO: 886 - DNA, 18 bp, synthetic construct
  source 1..18: mol_type = other DNA
gaaatcccatccctcgtc

SEQ ID NO: 887 - DNA, 20 bp, synthetic construct
  source 1..20: mol_type = other DNA
ccctactcctattccaccac

SEQ ID NO: 888 - DNA, 18 bp, synthetic construct
  source 1..18: mol_type = other DNA
gaaatcccatccctcgtc

SEQ ID NO: 889 - RNA, 23 nt, synthetic construct
  source 1..23: mol_type = other RNA
atatgaggtgaaaacactgcttt

SEQ ID NO: 890 - RNA, 23 nt, synthetic construct
  source 1..23: mol_type = other RNA
atatgaggtgaaaacactgctag

SEQ ID NO: 891 - RNA, 23 nt, synthetic construct
  source 1..23: mol_type = other RNA
atatgaggtgaaaacactgctat

SEQ ID NO: 892 - RNA, 23 nt, synthetic construct
  source 1..23: mol_type = other RNA
atatgaggtgaaaacactgccag

SEQ ID NO: 893 - RNA, 23 nt, synthetic construct
  source 1..23: mol_type = other RNA
atatgaggtgaaaacactgcgag

SEQ ID NO: 894 - RNA, 23 nt, synthetic construct
  source 1..23: mol_type = other RNA
atatgaggtgaaaacactgccgg

SEQ ID NO: 895 - RNA, 23 nt, synthetic construct
  source 1..23: mol_type = other RNA
atatgaggtgaaaacactgcggg

SEQ ID NO: 896 - RNA, 23 nt, synthetic construct
  source 1..23: mol_type = other RNA
taggtgaaaacactgctttagag

SEQ ID NO: 897 - RNA, 23 nt, synthetic construct
  source 1..23: mol_type = other RNA
taggtgaaaacactgctttagtg

SEQ ID NO: 898 - RNA, 23 nt, synthetic construct
  source 1..23: mol_type = other RNA
taggtgaaaacactgctttacgg

SEQ ID NO: 899 - RNA, 23 nt, synthetic construct
  source 1..23: mol_type = other RNA
taggtgaaaacactgctttacag

SEQ ID NO: 900 - RNA, 23 nt, synthetic construct
  source 1..23: mol_type = other RNA
taggtgaaaacactgctttatgg

SEQ ID NO: 901 - RNA, 23 nt, synthetic construct
  source 1..23: mol_type = other RNA
taggtgaaaacactgctttatag

SEQ ID NO: 902 - RNA, 21 nt, synthetic construct
  source 1..21: mol_type = other RNA
atatgaggtgaaaacactgct

SEQ ID NO: 903 - RNA, 21 nt, synthetic construct
  source 1..21: mol_type = other RNA
atatgaggtgaaaacactgag

SEQ ID NO: 904 - RNA, 21 nt, synthetic construct
  source 1..21: mol_type = other RNA
atatgaggtgaaaacacttag

SEQ ID NO: 905 - RNA, 21 nt, synthetic construct
  source 1..21: mol_type = other RNA
taggtgaaaacactgctttag

SEQ ID NO: 906 - RNA, 21 nt, synthetic construct
  source 1..21: mol_type = other RNA
taggtgaaaacactgctttgg

SEQ ID NO: 907 - RNA, 21 nt, synthetic construct
  source 1..21: mol_type = other RNA
ggcagtgttttcacctcatat

SEQ ID NO: 908 - RNA, 21 nt, synthetic construct
  source 1..21: mol_type = other RNA
cgcagtgttttcacctcatat

SEQ ID NO: 909 - RNA, 21 nt, synthetic construct
  source 1..21: mol_type = other RNA
gtaaagcagtgttttcaccta

SEQ ID NO: 910 - RNA, 21 nt, synthetic construct
  source 1..21: mol_type = other RNA
ataaagcagtgttttcaccta

SEQ ID NO: 911 - RNA, 19 nt, synthetic construct
  source 1..19: mol_type = other RNA
cagtgttttcacctcatat

SEQ ID NO: 912 - RNA, 19 nt, synthetic construct
  source 1..19: mol_type = other RNA
aagtgttttcacctcatat

SEQ ID NO: 913 - RNA, 19 nt, synthetic construct
  source 1..19: mol_type = other RNA
aaagcagtgttttcaccta

SEQ ID NO: 914 - RNA, 23 nt, synthetic construct
  source 1..23: mol_type = other RNA
atatgaggtgaaaacactgcttt

SEQ ID NO: 915 - RNA, 23 nt, synthetic construct
  source 1..23: mol_type = other RNA
atatgaggtgaaaacactgctat